European Patent Specification EP 3 434 764 B1, published April 8, 2026. Title: FABRIC & HOME CARE PRODUCTS. Applicant: The Procter & Gamble Company. The sequence listing filed with the application follows.

SEQUENCE LISTING (765 sequences)

SEQ ID NO: 1 - DNA, 1146 bp, Bacillus Amyloliquefaciens
gtgagaagcaaaaaattgtggatcagtttgctgtttgctttagcgttaatctttacgatggcgttcggcagcacatcctctgcccaggcggcagggaaatcaaacggggaaaagaaatatattgtcgggtttaaacagacaatgagcacgatgagcgccgctaagaagaaagatgtcatttctgaaaaaggcgggaaagtgcaaaagcaattcaaatatgtagacgcagcttcagctacattaaacgaaaaagctgtaaaagaattgaaaaaagacccgagcgtcgcttacgttgaagaagatcacgtagcacatgcgtacgcgcagtccgtgccttacggcgtatcacaaattaaagcccctgctctgcactctcaaggctacactggatcaaatgttaaagtagcggttatcgacagcggtatcgactcgagccatccagatcttaaagtcgctggaggggcttctatggtgccgtccgaaacaaacccgtttcaagataacaattctcatggcacacacgtcgcaggaacggttgcggcgttaaacaattctattggcgtgcttggtgtagccccgtctgcttcgctctacgccgttaaagttcttggcgcagacggatcaggccaatactcatggattatcaacggcatcgaatgggccatcgcgaataacatggatgtaatcaacatgagcctgggaggaccaagcggcagtgcggcacttaaagcagcagttgataaagctgttgcatctggtgtcgtcgtagtagcggcagctgggaatgagggaacatccggatcatcgagtaccgtcggttatccaggcaagtacccttcagtgattgcagtgggcgctgtagactcttcaaatcaacgtgcctctttttcctccgtgggaccggagctggatgtcatggcccctggcgtttctattcaatcgacgcttccagggaacaagtatggtgcgtataacgggacttccatggcctcgccgcatgtagctggggcggccgcattgattctttctaagcacccgaactggacaaacactcaagtccgcagcagtttagaaaacaccactacaaaacttggtgattctttctactatggaaaagggctgatcaacgtacaggcggcagctcag

SEQ ID NO: 2 - protein, 275 aa, Bacillus Amyloliquefaciens [sequence omitted]

SEQ ID NO: 3 - DNA, 825 bp, Artificial sequence
  Mutant of BPN'
gcgcagtccgtgccttacggcgtatcacaaattaaagcccctgctctgcactctcaaggctacactggatcaaatgttaaagtagcggttatcgacagcggtatcgactcgagccatccagatcttaaagtcgctggaggggcttctatggtgccgtccgaaacaaacccgtttcaagataacaattctcatggcacacacgtcgcaggaacggttgcggcgttaaacaattctattggcgtgcttggtgtagccccgtctgcttcgctctacgccgttaaagttcttgcagcagacggatcaggccaatactcatggattatcaacggcatcgaatgggccatcgcgaataacatggatgtaatcaacatgagcctgggagcaccaagcggcagtgcggcacttaaagcagcagttgataaagctgttgcatctggtgtcgtcgtagtagcggcagctgggaatgagggaacatccggatcatcgagtaccgtcggttatccaggcaagtacccttcagtgattgcagtgggcgctgtagactcttcaaatcaacgtgcctctttttcctccgtgggaccggagctggatgtcatggcccctggcgtttctattcaatcgacgcttccagggaacaagtatggtgcgcaaaacgggacttccatggcctcgccgcatgtagctggggcggccgcattgattctttctaagcacccgaactggacaaacactcaagtccgcagcagtttagaaaacaccactacaaaacttggtgattctttctactatggaaaagggctgatcaacgtacaggcggcagctcag

SEQ ID NO: 4 - protein, 275 aa, Artificial Sequence
  Mutant of subtilisin BPN'
AQSVPYGVSQIKAPALHSQGYTGSNVKVAVIDSGIDSSHPDLKVAGGASMVPSETNPFQDNNSHGTHVAGTVAALNNSIGVLGVAPSASLYAVKVLAADGSGQYSWIINGIEWAIANNMDVINMSLGAPSGSAALKAAVDKAVASGVVVVAAAGNEGTSGSSSTVGYPGKYPSVIAVGAVDSSNQRASFSSVGPELDVMAPGVSIQSTLPGNKYGAQNGTSMASPHVAGAAALILSKHPNWTNTQVRSSLENTTTKLGDSFYYGKGLINVQAAAQ

SEQ ID NO: 5 - DNA, 825 bp, Artificial Sequence
  Mutant of subtilisisn BPN'
gcgcagtccgtgccttacggcgtatcacaaattaaagcccctgctctgcactctcaaggctacactggaggcaatgttaaagtagcggttatcgacagcggtatcgactcgagccatccagatcttaaagtcgctggaggggcttctatggtgccgggcgaaacaaacccgtttcaagataacaattctcatggcacacacgtcgcaggaacggttgcggcgttaaacaataatattggcgtgcttggtgtagccccgtctgcttcgctctacgccgttaaagttcttggcgcagacggaaatggccaatactcatggattatcaacggcatcgaatgggccatcgcgaataacatggatgtaatcaacatgagcctgggagcaccaagcggcagtgcggcacttaaagcagcagttgataaagctgttgcatctggtgtcgtcgtagtagcggcagctgggaatgagggaacatccggatcatcgagtaccgtcggttatccaggcaagtacccttcagtgattgcagtgggcgctgtagactcttcaaatcaacgtgcctctttttcctccgtgggaccggagctggatgtcatggcccctggcgtttctattcaatcgacgcttccagggaacaagtatggtgcgcaaaacgggacttccatggcctcgccgcatgtagctggggcggccgcattgattctttctaagcacccgaactggacaaacactcaagtccgcagcagtttagaaaacaccactacaaaacttggtgattctttctactatggaaaagggctgatcaacgtacaggcggcagctcag

SEQ ID NO: 6 - protein, 275 aa, Artificial Sequence
  Mutant of subtilisin BPN'
AQSVPYGVSQIKAPALHSQGYTGGNVKVAVIDSGIDSSHPDLKVAGGASMVPGETNPFQDNNSHGTHVAGTVAALNNNIGVLGVAPSASLYAVKVLGADGNGQYSWIINGIEWAIANNMDVINMSLGAPSGSAALKAAVDKAVASGVVVVAAAGNEGTSGSSSTVGYPGKYPSVIAVGAVDSSNQRASFSSVGPELDVMAPGVSIQSTLPGNKYGAQNGTSMASPHVAGAAALILSKHPNWTNTQVRSSLENTTTKLGDSFYYGKGLINVQAAAQ

SEQ ID NO: 7 - DNA, 825 bp, Artificial Sequence
  Mutant of subtilisin BPN'
gcgcagtccgtgccttacggcgtatcacaaattaaagcccctgctctgcactctcaaggctacactggatcaaatgttaaagtagcggttatcgacagcggtattgattcgagccatccagatcttaaagtcgctggaggggcttctatggtgccgtccgaaacaaacccgtttcaagataacaattctcatggcacacacgtcgcaggaacggttgcggcgttaaacaataatattggcgtgcttggtgtagccccgtctgcttcgctctacgccgttaaagttcttgcagcagacggatcaggccaatactcatggattatcaacggcatcgaatgggccatcgcgaataacatggatgtaatcaacatgagcctgggagcaccaagcggcagtgcggcacttaaagcagcagttgataaagctgttgcatctggtgtcgtcgtagtagcggcagctgggaatgagggaacatccggatcatcgagtaccgtcggttatccaggcaagtacccttcagtgattgcagtgggcgctgtagactcttcaaatcaacgtgcctctttttcctccgtgggaccggagctggatgtcatggcccctggcgtttctattcaatcgacgcttccagggaacaagtatggtgcgcaaaacgggacttccatggcctcgccgcatgtagctggggcggccgcattgattctttctaagcacccgaactggacaaacactcaagtccgcagcagtttagaaaacaccactacaaaacttggtgattctttctactatggaaaagggctgatcaacgtacaggcggcagctcag

SEQ ID NO: 8 - protein, 275 aa, Artificial Sequence
  Mutant of subtilisin BPN'
AQSVPYGVSQIKAPALHSQGYTGSNVKVAVIDSGIDSSHPDLKVAGGASMVPSETNPFQDNNSHGTHVAGTVAALNNNIGVLGVAPSASLYAVKVLAADGSGQYSWIINGIEWAIANNMDVINMSLGAPSGSAALKAAVDKAVASGVVVVAAAGNEGTSGSSSTVGYPGKYPSVIAVGAVDSSNQRASFSSVGPELDVMAPGVSIQSTLPGNKYGAQNGTSMASPHVAGAAALILSKHPNWTNTQVRSSLENTTTKLGDSFYYGKGLINVQAAAQ

SEQ ID NO: 9 - DNA, 828 bp, Artificial Sequence
  Mutant of subtilisin BPN'
gcgcagtccgtgccttacggcgtatcacaaattaaagcccctgctctgcactctcaaggctacactggatcaaatgttaaagtagcggttatcgacagcggtatcgactcgagccatccagatcttaaagtcgctggaggggcttctatggtgccgggagaaacaaacccgtttcaagataacaattctcatggcacacacgcagcaggaacggttgcggcgttaaacaataatattggcgtgcttggtgtagccccgtctgcttcgctctacgccgttaaagttcttgcagcagacggatcagcacaatactcatggattatcaacggcatcgaatgggccatcgcgaataacatggatgtaatcaacatgagcctgggagcaacaagcggcagtgcggcacttaaagcagcagttgataaagctgttgcatctggtgtcgtcgtagtagcggcagctgggaatgagggaacatccggatcatcgagtaccgtcggttatccaggcaagtacccttcagtgattgcagtgggcgctgtagactcttcaaatacacgtgcctctttttcctccgtgggaccggagctggatgtcatggcccctggcgtttctattcaatcgacgcttccagggaacaagtatggtgcgcaaaacgggacttccatggcctcgccgcatgtagctggggcggccgcattgattctttctaagcacccgaactggacaaacactcaagtccgcagcagtttagaaaacaccactacaaaacttggtgattctttctactatggaaaagggctgatcaacgtacaggcggcagctcagtaa

SEQ ID NO: 10 - protein, 275 aa, Artificial Sequence
  Mutant of subtilisin BPN'
AQSVPYGVSQIKAPALHSQGYTGSNVKVAVIDSGIDSSHPDLKVAGGASMVPGETNPFQDNNSHGTHAAGTVAALNNNIGVLGVAPSASLYAVKVLAADGSAQYSWIINGIEWAIANNMDVINMSLGATSGSAALKAAVDKAVASGVVVVAAAGNEGTSGSSSTVGYPGKYPSVIAVGAVDSSNTRASFSSVGPELDVMAPGVSIQSTLPGNKYGAQNGTSMASPHVAGAAALILSKHPNWTNTQVRSSLENTTTKLGDSFYYGKGLINVQAAAQ

SEQ ID NO: 11 - DNA, 828 bp, Artificial Sequence
  Mutant of subtilisin BPN'
gcgcagtccgtgccttacggcgtatcacaaattaaagcccctgctctgcactctcaaggctacactggatcaaatgttaaagtagcggttatcgacagcggtatcgactcgagccatccagatcttaaagtcgctggaggggcttctatggtgccgtccgaaacaaacccgtttgtcgataacaattctcatggcacacacgtcgcaggaacggttgcggcgttaaacaataatattggcgtgcttggtgtagccccgtctgcttcgctctacgccgttaaagttcttgcagcagacggatcaggccaatactcatggattgtcaacggcatcgaatgggccatcgcgaataacatggatgtaatcaacatgagcctgggagcaccaagcggcagtgcggcacttaaagcagcagttgataaagctgttgcatctggtcaagtcgtagtagcggcagctgggaatgagggaacatccggatcatcgagtaccgtcggttatccaggcaagtacccttcagtgattgcagtgggcgctgtagactcttcaaatcaacgtgcctctttttcctccgtgggaccggagctggatgtcatggcccctggcgtttctattcaatcgacgcttccagcaaacaagtatggtgcgcaaaacgggacttccatggcctcgccgcatgtagctggggcggccgcattgattctttctaagcacccgaactggacaaacactcaagtccgcagcagtttagaacaaaccactacaaaacttggtgattctttctactatggaaaagggctgatcaacgtacaggcggcagctcagtaa

SEQ ID NO: 12 - protein, 275 aa, Artificial Sequence
  Mutant of subtilisin BPN'
AQSVPYGVSQIKAPALHSQGYTGSNVKVAVIDSGIDSSHPDLKVAGGASMVPSETNPFVDNNSHGTHVAGTVAALNNNIGVLGVAPSASLYAVKVLAADGSGQYSWIVNGIEWAIANNMDVINMSLGAPSGSAALKAAVDKAVASGQVVVAAAGNEGTSGSSSTVGYPGKYPSVIAVGAVDSSNQRASFSSVGPELDVMAPGVSIQSTLPANKYGAQNGTSMASPHVAGAAALILSKHPNWTNTQVRSSLEQTTTKLGDSFYYGKGLINVQAAAQ

SEQ ID NO: 13 - DNA, 828 bp, Artificial Sequence
  Mutant of subtilisin BPN'
gcgcagtccgtgccttacggcgtatcacaaattaaagcccctgctctgcactctcaaggctacactggatcaaatgttaaagtagcggttatcgacagcggtatcgactcgagccatccagatcttaaagtcgctggaggggcttctatggtgccgtccgaaacaaacccgtttcaagatgcaaattctcatggcacacacgtcgcaggaacggttgcggcgttaaacaataatattggcgtgcttggtgtagccccggaagcttcgctctacgccgttaaagttcttgcagcagacggatcaggccaatactcatggattatcaacggcatcgaatgggccatcgcgaataacatggatgtaatcaacatcagcctgggagcaccaagcggcagtgcggcacttaaagcagcagttgataaagctgttgcatctggtgtcgtcgtagtagcggcagctgggaatgagggaacatccggaccttcgagtaccgtcggttatccaggcaagtacccttcagtgattgcagtgggcgctgtagactcttcaaatcaacgtgcctctttttcctccgtgggaccggagctggatgtcatggcccctggcgtttctattcaatcgacgcttccagggaacaagtatggtgcgcaaaacgggacttccatggccgcaccgcatgtagctggggcggccgcattgattctttctaagcacccgaactggacaaacactcaagtccgcagcagtttagaaaacaccactacaaaacttggtgattctttctactatggaaaagggctgatcaacgtacaggcggcagctcagtaa

SEQ ID NO: 14 - protein, 275 aa, Artificial Sequence
  Mutant of subtilisn BPN'
AQSVPYGVSQIKAPALHSQGYTGSNVKVAVIDSGIDSSHPDLKVAGGASMVPSETNPFQDANSHGTHVAGTVAALNNNIGVLGVAPEASLYAVKVLAADGSGQYSWIINGIEWAIANNMDVINISLGAPSGSAALKAAVDKAVASGVVVVAAAGNEGTSGPSSTVGYPGKYPSVIAVGAVDSSNQRASFSSVGPELDVMAPGVSIQSTLPGNKYGAQNGTSMAAPHVAGAAALILSKHPNWTNTQVRSSLENTTTKLGDSFYYGKGLINVQAAAQ

SEQ ID NO: 15 - DNA, 828 bp, Artificial Sequence
  Mutant of subtilisin BPN'
gcgcagtccgtgccttacggcgtatcacaaattaaagcccctgctctgcactctcaaggctacactggatcaaatgttaaagtagcggttatcgacagcggtatcgactcgagccatccagatcttaaagtcgctggaggggcttctatggtgccgtccgaaacaaacccgtttcaagataaccaatctcatggcacacacgtcgcaggaacggttgcggcgttaaacaataatattggcgtgcttggtgtagccccgtctgcttcgctctacgccgttaaagttcttgcagcagacaactcaggccaatactcatggattatcaacggcatcgaatgggccatcgcgaataacatggatgtaatcaacatggcactgggagcaccaagcggcagtgcggcacttaaagcagcagttgataaagctgttgcatctggtgtcgtcgtagtagcggcagctgggaatgagggaacagatggatcatcgagtaccgtcggttatccaggcaagtacccttcagtgattgcagtgggcgctgtagactcttcaaatcaacgtgcctctttttcctccgtgggaccggagctggatgtcatggcccctggcgtttctattcaatcgacgcttccagggaacaagtatggtgcgcaaaacgggacttccatggcctcgccgcatgtagctggggcggccgcattgattctttctaagcacccgtcatggacaaacactcaagtccgcagcagtttagaaaacaccactacaaaacttggtgattctttctactatggaaaagggctgatcaacgtacaggcggcagctcagtaa

SEQ ID NO: 16 - protein, 275 aa, Artificial Sequence
  Mutant of subtilisin BPN'
AQSVPYGVSQIKAPALHSQGYTGSNVKVAVIDSGIDSSHPDLKVAGGASMVPSETNPFQDNQSHGTHVAGTVAALNNNIGVLGVAPSASLYAVKVLAADNSGQYSWIINGIEWAIANNMDVINMALGAPSGSAALKAAVDKAVASGVVVVAAAGNEGTDGSSSTVGYPGKYPSVIAVGAVDSSNQRASFSSVGPELDVMAPGVSIQSTLPGNKYGAQNGTSMASPHVAGAAALILSKHPSWTNTQVRSSLENTTTKLGDSFYYGKGLINVQAAAQ

SEQ ID NO: 17 - DNA, 828 bp, Artificial Sequence
  Mutant of subtilisin BPN'
gcgcagtccgtgccttacggcgtatcacaaattaaagcccctgctctgcactctcaaggctacactggatcaaatgttaaagtagcggttatcgacagcggtatcgactcgagccatccagatcttaaagtcgctggaggggcttctatggtgccgtccgaaacaaacccgtttcaagataacaatacacatggcacacacgtcgcaggaacggttgcggcgttaaacaataatattggcgtgcttggtgtagccccgtctgcttcgctctacgccgttaaagttcttgcagcagacggagcaggccaatactcatggattatcaacggcatcgaatgggccatcgcgaataacatggatgtaatcaacatgagcgtcggagcaccaagcggcagtgcggcacttaaagcagcagttgataaagctgttgcatctggtgtcgtcgtagtagcggcagctgggaatgagggaacatccggatcatcgagtaccgtcggttatccaggcaagtacccttcagtgattgcagtgggcgctgtagactctacaaatcaacgtgcctctttttcctccgtgggaccggagctggatgtcatggcccctggcgtttctattcaatcgacgcttccagggaacaagtatggtgcgcaaaacgggacttccatggcctcgccgcatgtagctggggcggccgcattgattctttctaagcacccgaactggacaaacaaccaagtccgcagcagtttagaaaacaccactacaaaacttggtgattctttctactatggaaaagggctgatcaacgtacaggcggcagctcagtaa

SEQ ID NO: 18 - protein, 275 aa, Artificial Sequence
  Mutant of subtilisin BPN'
AQSVPYGVSQIKAPALHSQGYTGSNVKVAVIDSGIDSSHPDLKVAGGASMVPSETNPFQDNNTHGTHVAGTVAALNNNIGVLGVAPSASLYAVKVLAADGAGQYSWIINGIEWAIANNMDVINMSVGAPSGSAALKAAVDKAVASGVVVVAAAGNEGTSGSSSTVGYPGKYPSVIAVGAVDSTNQRASFSSVGPELDVMAPGVSIQSTLPGNKYGAQNGTSMASPHVAGAAALILSKHPNWTNNQVRSSLENTTTKLGDSFYYGKGLINVQAAAQ

SEQ ID NO: 19 - DNA, 828 bp, Artificial Sequence
  Mutant of subtilisin BPN'
gcgcagtccgtgccttacggcgtatcacaaattaaagcccctgctctgcactctcaaggctacactggatcaaatgttaaagtagcggttatcgacagcggtatcgactcgagccatctggatcttaaagtcgctggaggggcttctatggtgccgggagaaacaaacccgtttgtcgatgcacaaacacatggcacacacgtcgcaggaacggttgcggcgttaaacaataatattggcgtgcttggtgtagccccggaagcttcgctctacgccgttaaagttcttgcagcagacaacgcagcacaatactcatggattgtcaacggcatcgaatgggccatcgcgaataacatggatgtaatcaacatgagcctgggagcaccaagcggcagtgcggcacttaaagcagcagttgataaagctgttgcatctggtgtcgtcgtagtagcggcagctgggaatgagggaacatccggatcatcgagtaccgtcggttatccaggcaagtacccttcagtgattgcagtgggcgctgtagactcttcaaatcaacgtgcctctttttcctccgtgggaccggagctggatgtcatggcccctggcgtttctattcaatcgacgcttccagggaacaagtatggtgcgcaaaacgggacttccatggcctcgccgcatgtagctggggcggccgcattgattctttctaagcacccgaactggacaaacactcaagtccgcagcagtttagaaaacaccactacaaaacttggtgattctttctactatggaaaagggctgatcaacgtacaggcggcagctcagtaa

SEQ ID NO: 20 - protein, 275 aa, Artificial Sequence
  Mutant of subtilisin BPN'
AQSVPYGVSQIKAPALHSQGYTGSNVKVAVIDSGIDSSHLDLKVAGGASMVPGETNPFVDAQTHGTHVAGTVAALNNNIGVLGVAPEASLYAVKVLAADNAAQYSWIVNGIEWAIANNMDVINMSLGAPSGSAALKAAVDKAVASGVVVVAAAGNEGTSGSSSTVGYPGKYPSVIAVGAVDSSNQRASFSSVGPELDVMAPGVSIQSTLPGNKYGAQNGTSMASPHVAGAAALILSKHPNWTNTQVRSSLENTTTKLGDSFYYGKGLINVQAAAQ

SEQ ID NO: 21 - DNA, 828 bp, Artificial Sequence
  Mutant of subtilisin BPN'
gcgcagtccgtgccttacggcgtatcacaaattaaagcccctgctctgcactctcaaggctacactggatcaaatgttaaagtagcggttatcgacagcggtatcgactcgagccatccagatcttaaagtcgctggaggggcttctatggtgccgtccgaaacaaacccgtttcaagataacaattctcatggcacacacgtcgcaggaacggttgcggcgttaaacaataatattggcgtgcttggtgtagccccgtctgcttcgctctacgccgttaaagttcttgcagcagacggatcaggccaatactcatggattatcaacggcatcgaatgggccatcgcgaataacatggatgtaatcaacatgagcctgggagcaacaagcggcagtgcggcacttaaagcagcagttgataaagctgttgcatctggtcaagtcgtagtagcggcagctgggaatgagggaacagatggaccttcgagtaccgtcggttatccaggcaagtacccttcagtgattgcagtgggcgctgtagactctacaaatacacgtgcctctttttcctccgtgggaccggagctggatgtcatggcccctggcgtttctattcaatcgacgcttccagcaaacaagtatggtgcgcaaaacgggacttccatggccgcaccgcatgtagctggggcggccgcattgattctttctaagcacccgtcatggacaaacaaccaagtccgcagcagtttagaacaaaccactacaaaacttggtgattctttctactatggaaaagggctgatcaacgtacaggcggcagctcagtaa

SEQ ID NO: 22 - protein, 275 aa, Artificial Sequence
  Mutant of subtilisin BPN'
AQSVPYGVSQIKAPALHSQGYTGSNVKVAVIDSGIDSSHPDLKVAGGASMVPSETNPFQDNNSHGTHVAGTVAALNNNIGVLGVAPSASLYAVKVLAADGSGQYSWIINGIEWAIANNMDVINMSLGATSGSAALKAAVDKAVASGQVVVAAAGNEGTDGPSSTVGYPGKYPSVIAVGAVDSTNTRASFSSVGPELDVMAPGVSIQSTLPANKYGAQNGTSMAAPHVAGAAALILSKHPSWTNNQVRSSLEQTTTKLGDSFYYGKGLINVQAAAQ

SEQ ID NO: 23 - DNA, 828 bp, Artificial Sequence
  Mutant of subtilisin BPN'
gcgcagtccgtgccttacggcgtatcacaaattaaagcccctgctctgcactctcaaggctacactggatcaaatgttaaagtagcggttatcgacagcggtatcgactcgagccatccagatcttaaagtcgctggaggggcttctatggtgccgtccgaaacaaacccgtttcaagataacaattctcatggcacacacgcagcaggaacggttgcggcgttaaacaataatattggcgtgcttggtgtagccccgtctgcttcgctctacgccgttaaagttcttgcagcagacggatcagcacaatactcatggattatcaacggcatcgaatgggccatcgcgaataacatggatgtaatcaacatggcactgggagcaccaagcggcagtgcggcacttaaagcagcagttgataaagctgttgcatctggtgtcgtcgtagtagcggcagctgggaatgagggaacatccggatcatcgagtaccgtcggttatccaggcaagtacccttcagtgattgcagtgggcgctgtagactcttcaaatcaacgtgcctctttttcctccgtgggaccggagctggatgtcatggcccctggcgtttctattcaatcgacgcttccagcaaacaagtatggtgcgcaaaacgggacttccatggcctcgccgcatgtagctggggcggccgcattgattctttctaagcacccgaactggacaaacactcaagtccgcagcagtttagaaaacaccactacaaaacttggtgattctttctactatggaaaagggctgatcaacgtacaggcggcagctcagtaa

SEQ ID NO: 24 - protein, 275 aa, Artificial Sequence
  Mutant of subtilisin BPN'
AQSVPYGVSQIKAPALHSQGYTGSNVKVAVIDSGIDSSHPDLKVAGGASMVPSETNPFQDNNSHGTHAAGTVAALNNNIGVLGVAPSASLYAVKVLAADGSAQYSWIINGIEWAIANNMDVINMALGAPSGSAALKAAVDKAVASGVVVVAAAGNEGTSGSSSTVGYPGKYPSVIAVGAVDSSNQRASFSSVGPELDVMAPGVSIQSTLPANKYGAQNGTSMASPHVAGAAALILSKHPNWTNTQVRSSLENTTTKLGDSFYYGKGLINVQAAAQ

SEQ ID NO: 25 - DNA, 36 bp, Artificial Sequence
  Primer
cttctatggtgccgtccgaaacaaacccgtttcaag

SEQ ID NO: 26 - DNA, 34 bp, Artificial Sequence
  Primer
tcatggcacacacgtcgcaggaacggttgcggcg

SEQ ID NO: 27 - DNA, 37 bp, Artificial Sequence
  Primer
agcagacggatcaggccaatactcatggattatcaac

SEQ ID NO: 28 - DNA, 39 bp, Artificial Sequence
  Primer
tgagcctgggagcaccaagcggcagtgcggcacttaaag

SEQ ID NO: 29 - DNA, 38 bp, Artificial Sequence
  Primer
tagactcttcaaatcaacgtgcctctttttcctccgtg

SEQ ID NO: 30 - DNA, 34 bp, Artificial Sequence
  Primer
gaaacaaacccgtttcaagataacaattctcatg

SEQ ID NO: 31 - DNA, 37 bp, Artificial Sequence
  Primer
atactcatggattatcaacggcatcgaatgggccatc

SEQ ID NO: 32 - DNA, 36 bp, Artificial Sequence
  Primer
tgttgcatctggtgtcgtcgtagtagcggcagctgg

SEQ ID NO: 33 - DNA, 37 bp, Artificial Sequence
  Primer
atcgacgcttccagggaacaagtatggtgcgcaaaac

SEQ ID NO: 34 - DNA, 35 bp, Artificial Sequence
  Primer
cagcagtttagaaaacaccactacaaaacttggtg

SEQ ID NO: 35 - DNA, 38 bp, Artificial Sequence
  Primer
caaacccgtttcaagataacaattctcatggcacacac

SEQ ID NO: 36 - DNA, 39 bp, Artificial Sequence
  Primer
ttggtgtagccccgtctgcttcgctctacgccgttaaag

SEQ ID NO: 37 - DNA, 36 bp, Artificial Sequence
  Primer
tggatgtaatcaacatgagcctgggagcaccaagcg

SEQ ID NO: 38 - DNA, 39 bp, Artificial Sequence
  Primer
agggaacatccggatcatcgagtaccgtcggttatccag

SEQ ID NO: 39 - DNA, 36 bp, Artificial Sequence
  Primer
gacttccatggcctcgccgcatgtagctggggcggc

SEQ ID NO: 40 - DNA, 36 bp, Artificial Sequence
  Primer
gtttcaagataacaattctcatggcacacacgtcgc

SEQ ID NO: 41 - DNA, 35 bp, Artificial Sequence
  Primer
gttcttgcagcagacggatcaggccaatactcatg

SEQ ID NO: 42 - DNA, 37 bp, Artificial Sequence
  Primer
atgtaatcaacatgagcctgggagcaccaagcggcag

SEQ ID NO: 43 - DNA, 37 bp, Artificial Sequence
  Primer
ggaatgagggaacatccggatcatcgagtaccgtcgg

SEQ ID NO: 44 - DNA, 38 bp, Artificial Sequence
  Primer
ctttctaagcacccgaactggacaaacactcaagtccg

SEQ ID NO: 45 - DNA, 36 bp, Artificial Sequence
  Primer
tcaagataacaattctcatggcacacacgtcgcagg

SEQ ID NO: 46 - DNA, 37 bp, Artificial Sequence
  Primer
tgcagcagacggatcaggccaatactcatggattatc

SEQ ID NO: 47 - DNA, 35 bp, Artificial Sequence
  Primer
aatcaacatgagcctgggagcaccaagcggcagtg

SEQ ID NO: 48 - DNA, 37 bp, Artificial Sequence
  Primer
cgctgtagactcttcaaatcaacgtgcctctttttcc

SEQ ID NO: 49 - DNA, 35 bp, Artificial Sequence
  Primer
gaactggacaaacactcaagtccgcagcagtttag

SEQ ID NO: 50 - DNA, 34 bp, Artificial Sequence; identical to SEQ ID NO: 26
  Primer

SEQ ID NO: 51 - DNA, 37 bp, Artificial Sequence; identical to SEQ ID NO: 27
  Primer

SEQ ID NO: 52 - DNA, 37 bp, Artificial Sequence; identical to SEQ ID NO: 33
  Primer

SEQ ID NO: 53 - DNA, 37 bp, Artificial Sequence; identical to SEQ ID NO: 42
  Primer

SEQ ID NO: 54 - DNA, 22 bp, Artificial Sequence
  Primer
tacatatgagttatgcagtttg

SEQ ID NO: 55 - DNA, 19 bp, Artificial Sequence
  Primer
ttatcctttaccttgtctc

SEQ ID NO: 56 - DNA, 35 bp, Artificial Sequence
  Primer
caacatgagcctgggatcaccaagcggcagtgcgg

SEQ ID NO: 57 - DNA, 35 bp, Artificial Sequence
  Primer
ccgcactgccgcttggtgatcccaggctcatgttg

SEQ ID NO: 58 - DNA, 38 bp, Artificial Sequence
  Primer
ctatggtgccgggcgaaacaaacccgtttcaagatccg

SEQ ID NO: 59 - DNA, 38 bp, Artificial Sequence
  Primer
cggatcttgaaacgggtttgtttcgcccggcaccatag

SEQ ID NO: 60 - DNA, 21 bp, Artificial Sequence
  Primer
gcctcacatttgtgccaccta

SEQ ID NO: 61 - DNA, 22 bp, Artificial Sequence
  Primer
cctctcggttatgagttagttc

SEQ ID NO: 62 - DNA, 24 bp, Artificial Sequence
  Primer
aaaggatcctaatcggcgcttttc

SEQ ID NO: 63 - DNA, 24 bp, Artificial Sequence
  Primer
cttgtctccaagcttaaaataaaa

SEQ ID NO: 64 - DNA, 36 bp, Artificial Sequence
  Primer
cagatcttaaagtctctggaggggcttctatggtgc

SEQ ID NO: 65 - DNA, 40 bp, Artificial Sequence
  Primer
catagaagcccctccagagactttaagatctggatggctc

SEQ ID NO: 66 - DNA, 36 bp, Artificial Sequence
  Primer
gcattgattctttacaagcacccgaactggacaaac

SEQ ID NO: 67 - DNA, 39 bp, Artificial Sequence
  Primer
cagttcgggtgcttgtaaagaatcaatgcggccgcccca

SEQ ID NO: 68 - DNA, 36 bp, Artificial Sequence
  Primer
gcattgattcttggtaagcacccgaactggacaaac

SEQ ID NO: 69 - DNA, 40 bp, Artificial Sequence
  Primer
ccagttcgggtgcttaccaagaatcaatgcggccgcccca

SEQ ID NO: 70 - DNA, 40 bp, Artificial Sequence
  Primer
catcgaatgggccacagcgaataacatggatgtaatcaac

SEQ ID NO: 71 - DNA, 40 bp, Artificial Sequence
  Primer
catccatgttattcgctgtggcccattcgatgccgttgat

SEQ ID NO: 72 - DNA, 40 bp, Artificial Sequence
  Primer
catcgaatgggccgtagcgaataacatggatgtaatcaac

SEQ ID NO: 73 - DNA, 40 bp, Artificial Sequence
  Primer
catccatgttattcgctacggcccattcgatgccgttgat

SEQ ID NO: 74 - DNA, 36 bp, Artificial Sequence
  Primer
ctgtagactctacaaatcaacgtgcctctttttcct

SEQ ID NO: 75 - DNA, 40 bp, Artificial Sequence
  Primer
aaagaggcacgttgatttgtagagtctacagcgcccactg

SEQ ID NO: 76 - DNA, 38 bp, Artificial Sequence
  Primer
ctgtagactcttcataccaacgtgcctctttttcctcc

SEQ ID NO: 77 - DNA, 40 bp, Artificial Sequence
  Primer
gaaaaagaggcacgttggtatgaagagtctacagcgccca

SEQ ID NO: 78 - DNA, 51 bp, Artificial Sequence
  Primer
tagcggttacagacagcggtatcgacccaagccatccagatcttaaagtcg

SEQ ID NO: 79 - DNA, 50 bp, Artificial Sequence
  Primer
atggcttgggtcgataccgctgtctgtaaccgctactttaacattgcctc

SEQ ID NO: 80 - DNA, 49 bp, Artificial Sequence
  Primer
taaagtagcggttacagacagcggtttagactcgagccatccagatctt

SEQ ID NO: 81 - DNA, 50 bp, Artificial Sequence
  Primer
atggctcgagtctaaaccgctgtctgtaaccgctactttaacattgcctc

SEQ ID NO: 82 - DNA, 50 bp, Artificial Sequence
  Primer
ggttgtagacagcggtatcgactcgtggcatccagatcttaaagtcgctg

SEQ ID NO: 83 - DNA, 50 bp, Artificial Sequence
  Primer
atgccacgagtcgataccgctgtctacaaccgctactttaacattgcctc

SEQ ID NO: 84 - DNA, 38 bp, Artificial Sequence
  Primer
ctacactggaggcaaagttaaagtagcggttatcgaca

SEQ ID NO: 85 - DNA, 40 bp, Artificial Sequence
  Primer
ataaccgctactttaactttgcctccagtgtagccttgag

SEQ ID NO: 86 - DNA, 37 bp, Artificial Sequence
  Primer
gagcctgggagcacgtagcggcagtgcggcacttaaa

SEQ ID NO: 87 - DNA, 40 bp, Artificial Sequence
  Primer
gtgccgcactgccgctacgtgctcccaggctcatgttgat

SEQ ID NO: 88 - DNA, 38 bp, Artificial Sequence
  Primer
tgagcctgggagcaaagagcggcagtgcggcacttaaa

SEQ ID NO: 89 - DNA, 38 bp, Artificial Sequence; identical to SEQ ID NO: 88
  Primer

SEQ ID NO: 90 - DNA, 40 bp, Artificial Sequence
  Primer
atcacaaattaaagccacagctctgcactctcaaggctac

SEQ ID NO: 91 - DNA, 40 bp, Artificial Sequence
  Primer
agagtgcagagctgtggctttaatttgtgatacgccgtaa

SEQ ID NO: 92 - DNA, 40 bp, Artificial Sequence; identical to SEQ ID NO: 91
  Primer

SEQ ID NO: 93 - DNA, 40 bp, Artificial Sequence
  Primer
taagatctggatggcttgtgtcgataccgctgtcgataac

SEQ ID NO: 94 - DNA, 40 bp, Artificial Sequence
  Primer
gacagcggtatcgacccaagccatccagatcttaaagtcg

SEQ ID NO: 95 - DNA, 40 bp, Artificial Sequence
  Primer
taagatctggatggcttgggtcgataccgctgtcgataac

SEQ ID NO: 96 - DNA, 40 bp, Artificial Sequence
  Primer
gacagcggtatcgactggagccatccagatcttaaagtcg

SEQ ID NO: 97 - DNA, 40 bp, Artificial Sequence
  Primer
taagatctggatggctccagtcgataccgctgtcgataac

SEQ ID NO: 98 - DNA, 40 bp, Artificial Sequence
  Primer
acgcgcagtccgtgttatacggcgtatcacaaattaaagc

SEQ ID NO: 99 - DNA, 40 bp, Artificial Sequence
  Primer
atttgtgatacgccgtataacacggactgcgcgtacgcat

SEQ ID NO: 100 - DNA, 37 bp, Artificial Sequence
  Primer
acaagtatggtgcgaaaaacgggacttccatggcctc

SEQ ID NO: 101 - DNA, 38 bp, Artificial Sequence
  Primer
catggaagtcccgtttttcgcaccatacttgttccctg

SEQ ID NO: 102 - DNA, 37 bp, Artificial Sequence
  Primer
acaagtatggtgcgggaaacgggacttccatggcctc

SEQ ID NO: 103 - DNA, 39 bp, Artificial Sequence
  Primer
ccatggaagtcccgtttcccgcaccatacttgttccctg

SEQ ID NO: 104 - DNA, 38 bp, Artificial Sequence
  Primer
cttacggcgtatcattaattaaagcccctgctctgcac

SEQ ID NO: 105 - DNA, 40 bp, Artificial Sequence
  Primer
gagcaggggctttaattaatgatacgccgtaaggcacgga

SEQ ID NO: 106 - DNA, 38 bp, Artificial Sequence
  Primer
cttacggcgtatcacgtattaaagcccctgctctgcac

SEQ ID NO: 107 - DNA, 40 bp, Artificial Sequence
  Primer
gagcaggggctttaatacgtgatacgccgtaaggcacgga

SEQ ID NO: 108 - DNA, 40 bp, Artificial Sequence
  Primer
tttagaaaacacctctacaaaacttggtgattctttctac

SEQ ID NO: 109 - DNA, 40 bp, Artificial Sequence
  Primer
tcaccaagttttgtagaggtgttttctaaactgctgcgga

SEQ ID NO: 110 - DNA, 40 bp, Artificial Sequence
  Primer
aggctacactggagcaaatgttaaagtagcggttatcgac

SEQ ID NO: 111 - DNA, 38 bp, Artificial Sequence
  Primer
gctactttaacatttgctccagtgtagccttgagagtg

SEQ ID NO: 112 - DNA, 39 bp, Artificial Sequence
  Primer
gagggaacatccggaccatcgagtaccgtcggttatcca

SEQ ID NO: 113 - DNA, 40 bp, Artificial Sequence
  Primer
accgacggtactcgatggtccggatgttccctcattccca

SEQ ID NO: 114 - DNA, 40 bp, Artificial Sequence
  Primer
agggaacatccggaccattaagtaccgtcggttatccagg

SEQ ID NO: 115 - DNA, 40 bp, Artificial Sequence
  Primer
accgacggtacttaatggtccggatgttccctcattccca

SEQ ID NO: 116 - DNA, 39 bp, Artificial Sequence
  Primer
gaacatccggatcattaagtaccgtcggttatccaggca

SEQ ID NO: 117 - DNA, 40 bp, Artificial Sequence
  Primer
ataaccgacggtacttaatgatccggatgttccctcattc

SEQ ID NO: 118 - DNA, 39 bp, Artificial Sequence
  Primer
gaacatccggatcaccaagtaccgtcggttatccaggca

SEQ ID NO: 119 - DNA, 40 bp, Artificial Sequence
  Primer
ataaccgacggtacttggtgatccggatgttccctcattc

SEQ ID NO: 120 - DNA, 38 bp, Artificial Sequence
  Primer
gtttagaaaacgcaactacaaaacttggtgattctttc

SEQ ID NO: 121 - DNA, 40 bp, Artificial Sequence
  Primer
caccaagttttgtagttgcgttttctaaactgctgcggac

SEQ ID NO: 122 - DNA, 40 bp, Artificial Sequence
  Primer
caaaacttggtgatccattctactatggaaaagggctgat

SEQ ID NO: 123 - DNA, 40 bp, Artificial Sequence
  Primer
tttccatagtagaatggatcaccaagttttgtagtggtgt

SEQ ID NO: 124 - DNA, 40 bp, Artificial Sequence
  Primer
caaaacttggtgataacttctactatggaaaagggctgat

SEQ ID NO: 125 - DNA, 40 bp, Artificial Sequence
  Primer
tttccatagtagaagttatcaccaagttttgtagtggtgt

SEQ ID NO: 126 - DNA, 40 bp, Artificial Sequence
  Primer
caaaacttggtgatatcttctactatggaaaagggctgat

SEQ ID NO: 127 - DNA, 40 bp, Artificial Sequence
  Primer
tttccatagtagaagatatcaccaagttttgtagtggtgt

SEQ ID NO: 128 - DNA, 40 bp, Artificial Sequence
  Primer
caaaacttggtgatggattctactatggaaaagggctgat

SEQ ID NO: 129 - DNA, 40 bp, Artificial Sequence
  Primer
tttccatagtagaatccatcaccaagttttgtagtggtgt

SEQ ID NO: 130 - DNA, 37 bp, Artificial Sequence
  Primer
gtgggcgctgtacactcttcaaatcaacgtgcctctt

SEQ ID NO: 131 - DNA, 40 bp, Artificial Sequence
  Primer
cacgttgatttgaagagtgtacagcgcccactgcaatcac

SEQ ID NO: 132 - DNA, 37 bp, Artificial Sequence
  Primer
gtgggcgctgtaggatcttcaaatcaacgtgcctctt

SEQ ID NO: 133 - DNA, 40 bp, Artificial Sequence
  Primer
cacgttgatttgaagatcctacagcgcccactgcaatcac

SEQ ID NO: 134 - DNA, 37 bp, Artificial Sequence
  Primer
cctgctctgcacttccaaggctacactggaggcaatg

SEQ ID NO: 135 - DNA, 40 bp, Artificial Sequence
  Primer
ctccagtgtagccttggaagtgcagagcaggggctttaat

SEQ ID NO: 136 - DNA, 37 bp, Artificial Sequence
  Primer
cctgctctgcacacacaaggctacactggaggcaatg

SEQ ID NO: 137 - DNA, 40 bp, Artificial Sequence
  Primer
ctccagtgtagccttgtgtgtgcagagcaggggctttaat

SEQ ID NO: 138 - DNA, 37 bp, Artificial Sequence
  Primer
cctgctctgcacccacaaggctacactggaggcaatg

SEQ ID NO: 139 - DNA, 40 bp, Artificial Sequence
  Primer
ctccagtgtagccttgtgggtgcagagcaggggctttaat

SEQ ID NO: 140 - DNA, 37 bp, Artificial Sequence
  Primer
cctgctctgcactaccaaggctacactggaggcaatg

SEQ ID NO: 141 - DNA, 40 bp, Artificial Sequence
  Primer
ctccagtgtagccttggtagtgcagagcaggggctttaat

SEQ ID NO: 142 - DNA, 37 bp, Artificial Sequence
  Primer
cctgctctgcacttacaaggctacactggaggcaatg

SEQ ID NO: 143 - DNA, 40 bp, Artificial Sequence
  Primer
ctccagtgtagccttgtaagtgcagagcaggggctttaat

SEQ ID NO: 144 - DNA, 38 bp, Artificial Sequence
  Primer
tgctctgcactctttaggctacactggaggcaatgtta

SEQ ID NO: 145 - DNA, 40 bp, Artificial Sequence
  Primer
ttgcctccagtgtagcctaaagagtgcagagcaggggctt

SEQ ID NO: 146 - DNA, 39 bp, Artificial Sequence
  Primer
atcgcgaataacatgaacgtaatcaacatgagcctggga

SEQ ID NO: 147 - DNA, 39 bp, Artificial Sequence
  Primer
ctcatgttgattacgttcatgttattcgcgatggcccat

SEQ ID NO: 148 - DNA, 37 bp, Artificial Sequence
  Primer
cttccagggaaccgttatggtgcgcaaaacgggactt

SEQ ID NO: 149 - DNA, 39 bp, Artificial Sequence
  Primer
gttttgcgcaccataacggttccctggaagcgtcgattg

SEQ ID NO: 150 - DNA, 40 bp, Artificial Sequence
  Primer
ctgcacttacaaggctctactggaggcaatgttaaagtag

SEQ ID NO: 151 - DNA, 49 bp, Artificial Sequence
  Primer
taacattgcctccagtagagccttgtaagtgcagagcaggggctttaat

SEQ ID NO: 152 - DNA, 43 bp, Artificial Sequence
  Primer
gctctgcacttacaaggcaacactggaggcaatgttaaagtag

SEQ ID NO: 153 - DNA, 48 bp, Artificial Sequence
  Primer
aacattgcctccagtgttgccttgtaagtgcagagcaggggctttaat

SEQ ID NO: 154 - DNA, 35 bp, Artificial Sequence
  Primer
cttacggcgtaacacaaattaaagcccctgctctg

SEQ ID NO: 155 - DNA, 38 bp, Artificial Sequence
  Primer
aggggctttaatttgtgttacgccgtaaggcacggact

SEQ ID NO: 156 - DNA, 40 bp, Artificial Sequence
  Primer
ttaaagcagcagttgatttcgctgttgcatctggtgtcgt

SEQ ID NO: 157 - DNA, 40 bp, Artificial Sequence
  Primer
agatgcaacagcgaaatcaactgctgctttaagtgccgca

SEQ ID NO: 158 - DNA, 40 bp, Artificial Sequence
  Primer
ttaaagcagcagttgatcgtgctgttgcatctggtgtcgt

SEQ ID NO: 159 - DNA, 40 bp, Artificial Sequence
  Primer
agatgcaacagcacgatcaactgctgctttaagtgccgca

SEQ ID NO: 160 - DNA, 40 bp, Artificial Sequence
  Primer
aaacccgtttcaagattctaattctcatggcacacacgtc

SEQ ID NO: 161 - DNA, 40 bp, Artificial Sequence
  Primer
tgtgccatgagaattagaatcttgaaacgggtttgtttcg

SEQ ID NO: 162 - DNA, 40 bp, Artificial Sequence
  Primer
aaacccgtttcaagatgataattctcatggcacacacgtc

SEQ ID NO: 163 - DNA, 40 bp, Artificial Sequence
  Primer
tgtgccatgagaattatcatcttgaaacgggtttgtttcg

SEQ ID NO: 164 - DNA, 39 bp, Artificial Sequence
  Primer
aagcggcagtgcgacacttaaagcagcagttgataaagc

SEQ ID NO: 165 - DNA, 40 bp, Artificial Sequence
  Primer
tcaactgctgctttaagtgtcgcactgccgcttggtgctc

SEQ ID NO: 166 - DNA, 37 bp, Artificial Sequence
  Primer
caagcggcagtgttgcacttaaagcagcagttgataa

SEQ ID NO: 167 - DNA, 40 bp, Artificial Sequence
  Primer
actgctgctttaagtgcaacactgccgcttggtgctccca

SEQ ID NO: 168 - protein, 382 aa, Bacillus Amyloliquefaciens
VRSKKLWISLLFALALIFTMAFGSTSSAQAAGKSNGEKKYIVGFKQTMSTMSAAKKKDVISEKGGKVQKQFKYVDAASATLNEKAVKELKKDPSVAYVEEDHVAHAYAQSVPYGVSQIKAPALHSQGYTGSNVKVAVIDSGIDSSHPDLKVAGGASMVPSETNPFQDNNSHGTHVAGTVAALNNSIGVLGVAPSASLYAVKVLGADGSGQYSWIINGIEWAIANNMDVINMSLGGPSGSAALKAAVDKAVASGVVVVAAAGNEGTSGSSSTVGYPGKYPSVIAVGAVDSSNQRASFSSVGPELDVMAPGVSIQSTLPGNKYGAYNGTSMASPHVAGAAALILSKHPNWTNTQVRSSLENTTTKLGDSFYYGKGLINVQAAAQ

SEQ ID NO: 169 - DNA, 36 bp, Artificial Sequence
  Primer
cggcgttaaacaataacattggcgtgcttggtgtag

SEQ ID NO: 170 - DNA, 37 bp, Artificial Sequence
  Primer
accaagcacgccaatgttattgtttaacgccgcaacc

SEQ ID NO: 171 - DNA, 39 bp, Artificial Sequence
  Primer
gtatcgactcgagccatgaagatcttaaagtcgctggag

SEQ ID NO: 172 - DNA, 38 bp, Artificial Sequence
  Primer
cagcgactttaagatcttcatggctcgagtcgataccg

SEQ ID NO: 173 - DNA, 39 bp, Artificial Sequence
  Primer
ttggtgtagccccggatgcttcgctctacgccgttaaag

SEQ ID NO: 174 - DNA, 35 bp, Artificial Sequence
  Primer
cgtagagcgaagcatccggggctacaccaagcacg

SEQ ID NO: 175 - DNA, 39 bp, Artificial Sequence
  Primer
gaacggttgcggcgttagataattctattggcgtgcttg

SEQ ID NO: 176 - DNA, 37 bp, Artificial Sequence
  Primer
agcacgccaatagaattatctaacgccgcaaccgttc

SEQ ID NO: 177 - DNA, 44 bp, Artificial Sequence
  Primer
aacggttgcggcgttagataataacattggcgtgcttggtgtag

SEQ ID NO: 178 - DNA, 46 bp, Artificial Sequence
  Primer
acaccaagcacgccaatgttattatctaacgccgcaaccgttcctg

SEQ ID NO: 179 - DNA, 31 bp, Artificial Sequence
  Primer
cggcgttaaacaataatattggcgtgcttgg

SEQ ID NO: 180 - DNA, 31 bp, Artificial Sequence
  Primer
ccaagcacgccaatattattgtttaacgccg

SEQ ID NO: 181 - DNA, 28 bp, Artificial Sequence
  Primer
ggtgtagccccggatgcttcgctctacg

SEQ ID NO: 182 - DNA, 28 bp, Artificial Sequence
  Primer
cgtagagcgaagcatccggggctacacc

SEQ ID NO: 183 - DNA, 30 bp, Artificial Sequence
  Primer
gtatcgactcgagccatgaagatcttaaag

SEQ ID NO: 184 - DNA, 30 bp, Artificial Sequence
  Primer
ctttaagatcttcatggctcgagtcgatac

SEQ ID NO: 185 - DNA, 28 bp, Artificial Sequence
  Primer
cgcttccagggaacaactatggtgcgta

SEQ ID NO: 186 - DNA, 28 bp, Artificial Sequence
  Primer
tacgcaccatagttgttccctggaagcg

SEQ ID NO: 187 - DNA, 31 bp, Artificial Sequence
  Primer
cactctcaaggctacgttggatcaaatgtta

SEQ ID NO: 188 - DNA, 31 bp, Artificial Sequence
  Primer
taacatttgatccaacgtagccttgagagtg

SEQ ID NO: 189 - DNA, 29 bp, Artificial Sequence
  Primer
tggcgtttctattgaatcgacgcttccag

SEQ ID NO: 190 - DNA, 29 bp, Artificial Sequence
  Primer
ctggaagcgtcgattcaatagaaacgcca

SEQ ID NO: 191 - DNA, 39 bp, Artificial Sequence; identical to SEQ ID NO: 175
  Primer

SEQ ID NO: 192 - DNA, 37 bp, Artificial Sequence; identical to SEQ ID NO: 176
  Primer

SEQ ID NO: 193 - DNA, 39 bp, Artificial Sequence; identical to SEQ ID NO: 173
  Primer

SEQ ID NO: 194 - DNA, 35 bp, Artificial Sequence; identical to SEQ ID NO: 174
  Primer

SEQ ID NO: 195 - DNA, 35 bp, Artificial Sequence
  Primer
gcagcagacggatcagcacaatactcatggattat

SEQ ID NO: 196 - DNA, 35 bp, Artificial Sequence
  Primer
ataatccatgagtattgtgctgatccgtctgctgc

SEQ ID NO: 197 - DNA, 45 bp, Artificial Sequence
  Primer
caacatgagcctgggagcaccaccgggcagtgcggcacttaaagc

SEQ ID NO: 198 - DNA, 45 bp, Artificial Sequence
  Primer
gctttaagtgccgcactgcccggtggtgctcccaggctcatgttg

SEQ ID NO: 199 - DNA, 39 bp, Artificial Sequence
  Primer
gttcttgcagcagacggaaatggccaatactcatggatt

SEQ ID NO: 200 - DNA, 39 bp, Artificial Sequence
  Primer
aatccatgagtattggccatttccgtctgctgcaagaac

SEQ ID NO: 201 - DNA, 42 bp, Artificial Sequence
  Primer
ttaaagttcttgcagcagacaattcaggccaatactcatgga

SEQ ID NO: 202 - DNA, 42 bp, Artificial Sequence
  Primer
tccatgagtattggcctgaattgtctgctgcaagaactttaa

SEQ ID NO: 203 - DNA, 36 bp, Artificial Sequence
  Primer
ccgtttcaagatccgaattctcatggcacacacgtc

SEQ ID NO: 204 - DNA, 38 bp, Artificial Sequence
  Primer
tgccatgagaattcggatcttgaaacgggtttgtttcg

SEQ ID NO: 205 - DNA, 40 bp, Artificial Sequence
  Primer
ttcaaatcaacgtgattctttttcctccgtgggaccggag

SEQ ID NO: 206 - DNA, 40 bp, Artificial Sequence
  Primer
acggaggaaaaagaatcacgttgatttgaagagtctacag

SEQ ID NO: 207 - DNA, 38 bp, Artificial Sequence
  Primer
caaatcaacgtgcctctgattcctccgtgggaccggag

SEQ ID NO: 208 - DNA, 38 bp, Artificial Sequence
  Primer
ctccggtcccacggaggaatcagaggcacgttgatttg

SEQ ID NO: 209 - DNA, 44 bp, Artificial Sequence
  Primer
agcggcagtgcggcacttaaagttgcagttgataaagctgttgc

SEQ ID NO: 210 - DNA, 44 bp, Artificial Sequence
  Primer
gcaacagctttatcaactgcaactttaagtgccgcactgccgct

SEQ ID NO: 211 - DNA, 39 bp, Artificial Sequence
  Primer
tcaagataacaatacacatggcacacacgtcgcaggaac

SEQ ID NO: 212 - DNA, 40 bp, Artificial Sequence
  Primer
acgtgtgtgccatgtgtattgttatcttgaaacgggtttg

SEQ ID NO: 213 - DNA, 40 bp, Artificial Sequence
  Primer
agacggatcaggcaattactcatggattatcaacggcatc

SEQ ID NO: 214 - DNA, 37 bp, Artificial Sequence
  Primer
taatccatgagtaattgcctgatccgtctgctgcaag

SEQ ID NO: 215 - DNA, 38 bp, Artificial Sequence
  Primer
acccgtttcaagataacgattctcatggcacacacgtc

SEQ ID NO: 216 - DNA, 38 bp, Artificial Sequence
  Primer
gacgtgtgtgccatgagaatcgttatcttgaaacgggt

SEQ ID NO: 217 - DNA, 37 bp, Artificial Sequence
  Primer
caatactcatggattatcgatggcatcgaatgggcca

SEQ ID NO: 218 - DNA, 37 bp, Artificial Sequence
  Primer
tggcccattcgatgccatcgataatccatgagtattg

SEQ ID NO: 219 - DNA, 39 bp, Artificial Sequence
  Primer
ctcttcaaatcaacgtgccgatttttcctccgtgggacc

SEQ ID NO: 220 - DNA, 39 bp, Artificial Sequence
  Primer
ggtcccacggaggaaaaatcggcacgttgatttgaagag

SEQ ID NO: 221 - DNA, 37 bp, Artificial Sequence
  Primer
caaacactcaagtccgcagaagtttagaaaacaccac

SEQ ID NO: 222 - DNA, 38 bp, Artificial Sequence
  Primer
gtgcttggtgtagccccgagagcttcgctctacgccgt

SEQ ID NO: 223 - DNA, 38 bp, Artificial Sequence
  Primer
acggcgtagagcgaagctctcggggctacaccaagcac

SEQ ID NO: 224 - DNA, 37 bp, Artificial Sequence
  Primer
caaacactcaagtccgcgatagtttagaaaacaccac

SEQ ID NO: 225 - DNA, 37 bp, Artificial Sequence
  Primer
gtggtgttttctaaactatcgcggacttgagtgtttg

SEQ ID NO: 226 - DNA, 38 bp, Artificial Sequence
  Primer
gtgcttggtgtagccccgtctgcttcgctctacgccgt

SEQ ID NO: 227 - DNA, 38 bp, Artificial Sequence
  Primer
acggcgtagagcgaagcagacggggctacaccaagcac

SEQ ID NO: 228 - DNA, 37 bp, Artificial Sequence
  Primer
caatactcatggattatcaacggcatcgaatgggcca

SEQ ID NO: 229 - DNA, 37 bp, Artificial Sequence
  Primer
tggcccattcgatgccgttgataatccatgagtattg

SEQ ID NO: 230 - DNA, 37 bp, Artificial Sequence
  Primer
actcatggattatcgatggcatcgaatgggccatcgc

SEQ ID NO: 231 - DNA, 36 bp, Artificial Sequence
  Primer
cactcaagtccgcagaagtttagaaaacaccactac

SEQ ID NO: 232 - DNA, 36 bp, Artificial Sequence
  Primer
cactcaagtccgcgatagtttagaaaacaccactac

SEQ ID NO: 233 - DNA, 38 bp, Artificial Sequence
  Primer
caaatcaacgtgccagattttcctccgtgggaccggag

SEQ ID NO: 234 - DNA, 24 bp, Artificial Sequence
  Primer
aaaggggaggaaaatcgtgaaaca

SEQ ID NO: 235 - DNA, 22 bp, Artificial Sequence
  Primer
gttctaaatcgtgtttttcttg

SEQ ID NO: 236 - DNA, 48 bp, Artificial Sequence
  Primer
gaactggacaaacactcaagtccgcgatagtttagaaaacaccactac

SEQ ID NO: 237 - DNA, 36 bp, Artificial Sequence
  Primer
gacttgagtgtttgtccagttcgggtgcttagaaag

SEQ ID NO: 238 - DNA, 37 bp, Artificial Sequence
  Primer
caaacactcaagtccgcagcagtttagaaaacaccac

SEQ ID NO: 239 - DNA, 37 bp, Artificial Sequence
  Primer
gtggtgttttctaaactgctgcggacttgagtgtttg

SEQ ID NO: 240 - DNA, 49 bp, Artificial Sequence
  Primer
acgccgttaaagttcttgcagcagacgaatcaggccaatactcatggat

SEQ ID NO: 241 - DNA, 36 bp, Artificial Sequence
  Primer
tgctgcaagaactttaacggcgtagagcgaagcaga

SEQ ID NO: 242 - DNA, 37 bp, Artificial Sequence
  Primer
acatggatgtaatctgcatgagcctgggaggaccaag

SEQ ID NO: 243 - DNA, 38 bp, Artificial Sequence
  Primer
tcctcccaggctcatgcagattacatccatgttattcg

SEQ ID NO: 244 - DNA, 22 bp, Artificial Sequence
  Primer
gttatgagttagttcaaattcg

SEQ ID NO: 245 - DNA, 46 bp, Artificial Sequence
  Primer
  misc_feature (16)..(17): n is a, c, g, or t
  misc_feature (19)..(20): n is a, c, g, or t
  misc_feature (22)..(23): n is a, c, g, or t
tacgcgcagtccgtgnntnncnncgtatcacaaattaaagcccctg

SEQ ID NO: 246 - DNA, 44 bp, Artificial Sequence
  Primer
  misc_feature (17)..(18): n is a, c, g, or t
  misc_feature (20)..(21): n is a, c, g, or t
  misc_feature (23)..(24): n is a, c, g, or t
tttaatttgtgatacgnngnnanncacggactgcgcgtacgcat

SEQ ID NO: 247 - DNA, 43 bp, Artificial Sequence
  Primer
  misc_feature (16)..(17): n is a, c, g, or t
  misc_feature (19)..(20): n is a, c, g, or t
  misc_feature (22)..(23): n is a, c, g, or t
tacggcgtatcacaanntnnannccctgctctgcactctcaag

SEQ ID NO: 248 - DNA, 45 bp, Artificial Sequence
  Primer
  misc_feature (17)..(18): n is a, c, g, or t
  misc_feature (20)..(21): n is a, c, g, or t
  misc_feature (23)..(24): n is a, c, g, or t
agagtgcagagcagggnntnnannttgtgatacgccgtaaggcac

SEQ ID NO: 249 - DNA, 47 bp, Artificial Sequence
  Primer
  misc_feature (16)..(17): n is a, c, g, or t
  misc_feature (19)..(20): n is a, c, g, or t
  misc_feature (22)..(23): n is a, c, g, or t
gctctgcactctcaanncnncnntggatcaaatgttaaagtagcggt

SEQ ID NO: 250 - DNA, 47 bp, Artificial Sequence
  Primer
  misc_feature (17)..(18): n is a, c, g, or t
  misc_feature (20)..(21): n is a, c, g, or t
  misc_feature (23)..(24): n is a, c, g, or t
tttaacatttgatccanngnngnnttgagagtgcagagcaggggctt

SEQ ID NO: 251 - DNA, 48 bp, Artificial Sequence
  Primer
  misc_feature (16)..(17): n is a, c, g, or t
  misc_feature (19)..(20): n is a, c, g, or t
  misc_feature (22)..(23): n is a, c, g, or t
ctgcactctcaaggcnncnntnnatcaaatgttaaagtagcggttatc

SEQ ID NO: 252 - DNA, 44 bp, Artificial Sequence
  Primer
  misc_feature (17)..(18): n is a, c, g, or t
  misc_feature (20)..(21): n is a, c, g, or t
  misc_feature (23)..(24): n is a, c, g, or t
tactttaacatttgatnnanngnngccttgagagtgcagagcag

SEQ ID NO: 253 - DNA, 47 bp, Artificial Sequence
  Primer
  misc_feature (16)..(17): n is a, c, g, or t
  misc_feature (19)..(20): n is a, c, g, or t
  misc_feature (22)..(23): n is a, c, g, or t
cactctcaaggctacnntnnannaaatgttaaagtagcggttatcga

SEQ ID NO: 254 - DNA, 44 bp, Artificial Sequence
  Primer
  misc_feature (17)..(18): n is a, c, g, or t
  misc_feature (20)..(21): n is a, c, g, or t
  misc_feature (23)..(24): n is a, c, g, or t
cgctactttaacatttnntnnanngtagccttgagagtgcagag

SEQ ID NO: 255 - DNA, 46 bp, Artificial Sequence
  Primer
  misc_feature (16)..(17): n is a, c, g, or t
  misc_feature (19)..(20): n is a, c, g, or t
  misc_feature (22)..(23): n is a, c, g, or t
tctcaaggctacactnnannanntgttaaagtagcggttatcgaca

SEQ ID NO: 256 - DNA, 45 bp, Artificial Sequence
  Primer
  misc_feature (17)..(18): n is a, c, g, or t
  misc_feature (20)..(21): n is a, c, g, or t
  misc_feature (23)..(24): n is a, c, g, or t
aaccgctactttaacanntnntnnagtgtagccttgagagtgcag

SEQ ID NO: 257 - DNA, 45 bp, Artificial Sequence
  Primer
  misc_feature (16)..(17): n is a, c, g, or t
  misc_feature (19)..(20): n is a, c, g, or t
  misc_feature (22)..(23): n is a, c, g, or t
caaggctacactggannanntnntaaagtagcggttatcgacagc

SEQ ID NO: 258 - DNA, 45 bp, Artificial Sequence
  Primer
  misc_feature (17)..(18): n is a, c, g, or t
  misc_feature (20)..(21): n is a, c, g, or t
  misc_feature (23)..(24): n is a, c, g, or t
gataaccgctactttannanntnntccagtgtagccttgagagtg

SEQ ID NO: 259 - DNA, 45 bp, Artificial Sequence
  Primer
  misc_feature (16)..(17): n is a, c, g, or t
  misc_feature (19)..(20): n is a, c, g, or t
  misc_feature (22)..(23): n is a, c, g, or t
ggctacactggatcanntnntnnagtagcggttatcgacagcggt

SEQ ID NO: 260 - DNA, 45 bp, Artificial Sequence
  Primer
  misc_feature (17)..(18): n is a, c, g, or t
  misc_feature (20)..(21): n is a, c, g, or t
  misc_feature (23)..(24): n is a, c, g, or t
gtcgataaccgctactnnannanntgatccagtgtagccttgaga

SEQ ID NO: 261 - DNA, 44 bp, Artificial Sequence
  Primer
  misc_feature (16)..(17): n is a, c, g, or t
  misc_feature (19)..(20): n is a, c, g, or t
  misc_feature (22)..(23): n is a, c, g, or t
tacactggatcaaatnntnnannagcggttatcgacagcggtat

SEQ ID NO: 262 - DNA, 46 bp, Artificial Sequence
  Primer
  misc_feature (17)..(18): n is a, c, g, or t
  misc_feature (20)..(21): n is a, c, g, or t
  misc_feature (23)..(24): n is a, c, g, or t
gctgtcgataaccgctnntnnannatttgatccagtgtagccttga

SEQ ID NO: 263 - DNA, 45 bp, Artificial Sequence
  Primer
  misc_feature (16)..(17): n is a, c, g, or t
  misc_feature (19)..(20): n is a, c, g, or t
  misc_feature (22)..(23): n is a, c, g, or t
actggatcaaatgttnnannannggttatcgacagcggtatcgac

SEQ ID NO: 264 - DNA, 46 bp, Artificial Sequence
  Primer
  misc_feature (17)..(18): n is a, c, g, or t
  misc_feature (20)..(21): n is a, c, g, or t
  misc_feature (23)..(24): n is a, c, g, or t
accgctgtcgataaccnntnntnnaacatttgatccagtgtagcct

SEQ ID NO: 265 - DNA, 44 bp, Artificial Sequence
  Primer
  misc_feature (16)..(17): n is a, c, g, or t
  misc_feature (19)..(20): n is a, c, g, or t
  misc_feature (22)..(23): n is a, c, g, or t
ggatcaaatgttaaannanngnntatcgacagcggtatcgactc

SEQ ID NO: 266 - DNA, 47 bp, Artificial Sequence
  Primer
  misc_feature (17)..(18): n is a, c, g, or t
  misc_feature (20)..(21): n is a, c, g, or t
  misc_feature (23)..(24): n is a, c, g, or t
gataccgctgtcgatanncnntnntttaacatttgatccagtgtagc

SEQ ID NO: 267 - DNA, 48 bp, Artificial Sequence
  Primer
  misc_feature (16)..(17): n is a, c, g, or t
  misc_feature (19)..(20): n is a, c, g, or t
  misc_feature (22)..(23): n is a, c, g, or t
tcaaatgttaaagtanngnntnncgacagcggtatcgactcgagccat

SEQ ID NO: 268 - DNA, 48 bp, Artificial Sequence
  Primer
  misc_feature (17)..(18): n is a, c, g, or t
  misc_feature (20)..(21): n is a, c, g, or t
  misc_feature (23)..(24): n is a, c, g, or t
gtcgataccgctgtcgnnanncnntactttaacatttgatccagtgta

SEQ ID NO: 269 - DNA, 45 bp, Artificial Sequence
  Primer
  misc_feature (16)..(17): n is a, c, g, or t
  misc_feature (19)..(20): n is a, c, g, or t
  misc_feature (22)..(23): n is a, c, g, or t
aatgttaaagtagcgnntnncnncagcggtatcgactcgagccat

SEQ ID NO: 270 - DNA, 47 bp, Artificial Sequence
  Primer
  misc_feature (17)..(18): n is a, c, g, or t
  misc_feature (20)..(21): n is a, c, g, or t
  misc_feature (23)..(24): n is a, c, g, or t
cgagtcgataccgctgnngnnanncgctactttaacatttgatccag

SEQ ID NO: 271 - DNA, 45 bp, Artificial Sequence
  Primer
  misc_feature (16)..(17): n is a, c, g, or t
  misc_feature (19)..(20): n is a, c, g, or t
  misc_feature (22)..(23): n is a, c, g, or t
gttaaagtagcggttnncnncnncggtatcgactcgagccatcca

SEQ ID NO: 272 - DNA, 47 bp, Artificial Sequence
  Primer
  misc_feature (17)..(18): n is a, c, g, or t
  misc_feature (20)..(21): n is a, c, g, or t
  misc_feature (23)..(24): n is a, c, g, or t
gctcgagtcgataccgnngnngnnaaccgctactttaacatttgatc

SEQ ID NO: 273 - DNA, 45 bp, Artificial Sequence
  Primer
  misc_feature (16)..(17): n is a, c, g, or t
  misc_feature (19)..(20): n is a, c, g, or t
  misc_feature (22)..(23): n is a, c, g, or t
aaagtagcggttatcnncnncnntatcgactcgagccatccagat

SEQ ID NO: 274 - DNA, 47 bp, Artificial Sequence
  Primer
  misc_feature (17)..(18): n is a, c, g, or t
  misc_feature (20)..(21): n is a, c, g, or t
  misc_feature (23)..(24): n is a, c, g, or t
atggctcgagtcgatanngnngnngataaccgctactttaacatttg

SEQ ID NO: 275 - DNA, 44 bp, Artificial Sequence
  Primer
  misc_feature (16)..(17): n is a, c, g, or t
  misc_feature (19)..(20): n is a, c, g, or t
  misc_feature (22)..(23): n is a, c, g, or t
gtagcggttatcgacnncnntnncgactcgagccatccagatct

SEQ ID NO: 276 - DNA, 46 bp, Artificial Sequence
  Primer
  misc_feature (17)..(18): n is a, c, g, or t
  misc_feature (20)..(21): n is a, c, g, or t
  misc_feature (23)..(24): n is a, c, g, or t
tggatggctcgagtcgnnanngnngtcgataaccgctactttaaca

SEQ ID NO: 277 - DNA, 46 bp, Artificial Sequence
  Primer
  misc_feature (16)..(17): n is a, c, g, or t
  misc_feature (19)..(20): n is a, c, g, or t
  misc_feature (22)..(23): n is a, c, g, or t
gcggttatcgacagcnntnncnnctcgagccatccagatcttaaag

SEQ ID NO: 278 - DNA, 45 bp, Artificial Sequence
  Primer
  misc_feature (17)..(18): n is a, c, g, or t
  misc_feature (20)..(21): n is a, c, g, or t
  misc_feature (23)..(24): n is a, c, g, or t
atctggatggctcgagnngnnanngctgtcgataaccgctacttt

SEQ ID NO: 279 - DNA, 45 bp, Artificial Sequence
  Primer
  misc_feature (16)..(17): n is a, c, g, or t
  misc_feature (19)..(20): n is a, c, g, or t
  misc_feature (22)..(23): n is a, c, g, or t
gttatcgacagcggtnncnncnngagccatccagatcttaaagtc

SEQ ID NO: 280 - DNA, 44 bp, Artificial Sequence
  Primer
  misc_feature (17)..(18): n is a, c, g, or t
  misc_feature (20)..(21): n is a, c, g, or t
  misc_feature (23)..(24): n is a, c, g, or t
aagatctggatggctcnngnngnnaccgctgtcgataaccgcta

SEQ ID NO: 281 - DNA, 46 bp, Artificial Sequence
  Primer
  misc_feature (16)..(17): n is a, c, g, or t
  misc_feature (19)..(20): n is a, c, g, or t
  misc_feature (22)..(23): n is a, c, g, or t
atcgacagcggtatcnncnngnnccatccagatcttaaagtcgctg

SEQ ID NO: 282 - DNA, 47 bp, Artificial Sequence
  Primer
  misc_feature (17)..(18): n is a, c, g, or t
  misc_feature (20)..(21): n is a, c, g, or t
  misc_feature (23)..(24): n is a, c, g, or t
tttaagatctggatggnncnngnngataccgctgtcgataaccgcta

SEQ ID NO: 283 - DNA, 45 bp, Artificial Sequence
  Primer
  misc_feature (16)..(17): n is a, c, g, or t
  misc_feature (19)..(20): n is a, c, g, or t
  misc_feature (22)..(23): n is a, c, g, or t
gacagcggtatcgacnngnncnntccagatcttaaagtcgctgga

SEQ ID NO: 284 - DNA, 45 bp, Artificial Sequence
  Primer
  misc_feature (17)..(18): n is a, c, g, or t
  misc_feature (20)..(21): n is a, c, g, or t
  misc_feature (23)..(24): n is a, c, g, or t
gactttaagatctgganngnncnngtcgataccgctgtcgataac

SEQ ID NO: 285 - DNA, 44 bp, Artificial Sequence
  Primer
  misc_feature (16)..(17): n is a, c, g, or t
  misc_feature (19)..(20): n is a, c, g, or t
  misc_feature (22)..(23): n is a, c, g, or t
agcggtatcgactcgnncnntnnagatcttaaagtcgctggagg

SEQ ID NO: 286 - DNA, 44 bp, Artificial Sequence
  Primer
  misc_feature (17)..(18): n is a, c, g, or t
  misc_feature (20)..(21): n is a, c, g, or t
  misc_feature (23)..(24): n is a, c, g, or t
agcgactttaagatctnnanngnncgagtcgataccgctgtcga

SEQ ID NO: 287 - DNA, 44 bp, Artificial Sequence
  Primer
  misc_feature (16)..(17): n is a, c, g, or t
  misc_feature (19)..(20): n is a, c, g, or t
  misc_feature (22)..(23): n is a, c, g, or t
gactcgagccatccanntnntnnagtcgctggaggggcttctat

SEQ ID NO: 288 - DNA, 44 bp, Artificial Sequence
  Primer
  misc_feature (17)..(18): n is a, c, g, or t
  misc_feature (20)..(21): n is a, c, g, or t
  misc_feature (23)..(24): n is a, c, g, or t
agcccctccagcgactnnannanntggatggctcgagtcgatac

SEQ ID NO: 289 - DNA, 46 bp, Artificial Sequence
  Primer
  misc_feature (16)..(17): n is a, c, g, or t
  misc_feature (19)..(20): n is a, c, g, or t
  misc_feature (22)..(23): n is a, c, g, or t
agccatccagatcttnnanncnntggaggggcttctatggtgccgt

SEQ ID NO: 290 - DNA, 47 bp, Artificial Sequence
  Primer
  misc_feature (16)..(16): n is a, c, g, or t
  misc_feature (26)..(26): n is a, c, g, or t
catagaagcccctccnagcgactttnaagatctggatggctcgagtc

SEQ ID NO: 291 - DNA, 43 bp, Artificial Sequence
  Primer
  misc_feature (16)..(17): n is a, c, g, or t
  misc_feature (19)..(20): n is a, c, g, or t
  misc_feature (22)..(23): n is a, c, g, or t
catccagatcttaaanncnntnnaggggcttctatggtgccgt

SEQ ID NO: 292 - DNA, 46 bp, Artificial Sequence
  Primer
  misc_feature (17)..(18): n is a, c, g, or t
  misc_feature (20)..(21): n is a, c, g, or t
  misc_feature (23)..(24): n is a, c, g, or t
caccatagaagcccctnnanngnntttaagatctggatggctcgag

SEQ ID NO: 293 - DNA, 47 bp, Artificial Sequence
  Primer
  misc_feature (16)..(17): n is a, c, g, or t
  misc_feature (19)..(20): n is a, c, g, or t
  misc_feature (22)..(23): n is a, c, g, or t
ggaggggcttctatgnngnngnncgaaacaaacccgtttcaagataa

SEQ ID NO: 294 - DNA, 44 bp, Artificial Sequence
  Primer
  misc_feature (17)..(18): n is a, c, g, or t
  misc_feature (20)..(21): n is a, c, g, or t
  misc_feature (23)..(24): n is a, c, g, or t
aaacgggtttgtttcgnncnncnncatagaagcccctccagcga

SEQ ID NO: 295 - DNA, 47 bp, Artificial Sequence
  Primer
  misc_feature (16)..(17): n is a, c, g, or t
  misc_feature (19)..(20): n is a, c, g, or t
  misc_feature (22)..(23): n is a, c, g, or t
ggggcttctatggtgnngnncnnaacaaacccgtttcaagataacaa

SEQ ID NO: 296 - DNA, 44 bp, Artificial Sequence
  Primer
  misc_feature (17)..(18): n is a, c, g, or t
  misc_feature (20)..(21): n is a, c, g, or t
  misc_feature (23)..(24): n is a, c, g, or t
ttgaaacgggtttgttnngnncnncaccatagaagcccctccag

SEQ ID NO: 297 - DNA, 47 bp, Artificial Sequence
  Primer
  misc_feature (16)..(17): n is a, c, g, or t
  misc_feature (19)..(20): n is a, c, g, or t
  misc_feature (22)..(23): n is a, c, g, or t
gcttctatggtgccgnncnnannaaacccgtttcaagataacaattc

SEQ ID NO: 298 - DNA, 44 bp, Artificial Sequence
  Primer
  misc_feature (17)..(18): n is a, c, g, or t
  misc_feature (20)..(21): n is a, c, g, or t
  misc_feature (23)..(24): n is a, c, g, or t
atcttgaaacgggtttnntnngnncggcaccatagaagcccctc

SEQ ID NO: 299 - DNA, 47 bp, Artificial Sequence
  Primer
  misc_feature (16)..(17): n is a, c, g, or t
  misc_feature (19)..(20): n is a, c, g, or t
  misc_feature (22)..(23): n is a, c, g, or t
tctatggtgccgtccnnannanncccgtttcaagataacaattctca

SEQ ID NO: 300 - DNA, 46 bp, Artificial Sequence
  Primer
  misc_feature (17)..(18): n is a, c, g, or t
  misc_feature (20)..(21): n is a, c, g, or t
  misc_feature (23)..(24): n is a, c, g, or t
gttatcttgaaacgggnntnntnnggacggcaccatagaagcccct

SEQ ID NO: 301 - DNA, 47 bp, Artificial Sequence
  Primer
  misc_feature (16)..(17): n is a, c, g, or t
  misc_feature (19)..(20): n is a, c, g, or t
  misc_feature (22)..(23): n is a, c, g, or t
atggtgccgtccgaannanncnngtttcaagataacaattctcatgg

SEQ ID NO: 302 - DNA, 44 bp, Artificial Sequence
  Primer
  misc_feature (17)..(18): n is a, c, g, or t
  misc_feature (20)..(21): n is a, c, g, or t
  misc_feature (23)..(24): n is a, c, g, or t
attgttatcttgaaacnngnntnnttcggacggcaccatagaag

SEQ ID NO: 303 - DNA, 47 bp, Artificial Sequence
  Primer
  misc_feature (16)..(17): n is a, c, g, or t
  misc_feature (19)..(20): n is a, c, g, or t
  misc_feature (22)..(23): n is a, c, g, or t
gtgccgtccgaaacanncnngnntcaagataacaattctcatggcac

SEQ ID NO: 304 - DNA, 45 bp, Artificial Sequence
  Primer
  misc_feature (17)..(18): n is a, c, g, or t
  misc_feature (20)..(21): n is a, c, g, or t
  misc_feature (23)..(24): n is a, c, g, or t
agaattgttatcttganncnngnntgtttcggacggcaccataga

SEQ ID NO: 305 - DNA, 46 bp, Artificial Sequence
  Primer
  misc_feature (16)..(17): n is a, c, g, or t
  misc_feature (19)..(20): n is a, c, g, or t
  misc_feature (22)..(23): n is a, c, g, or t
ccgtccgaaacaaacnngnntnnagataacaattctcatggcacac

SEQ ID NO: 306 - DNA, 44 bp, Artificial Sequence
  Primer
  misc_feature (17)..(18): n is a, c, g, or t
  misc_feature (20)..(21): n is a, c, g, or t
  misc_feature (23)..(24): n is a, c, g, or t
atgagaattgttatctnnanncnngtttgtttcggacggcacca

SEQ ID NO: 307 - DNA, 45 bp, Artificial Sequence
  Primer
  misc_feature (16)..(17): n is a, c, g, or t
  misc_feature (19)..(20): n is a, c, g, or t
  misc_feature (22)..(23): n is a, c, g, or t
tccgaaacaaacccgnntnnanntaacaattctcatggcacacac

SEQ ID NO: 308 - DNA, 44 bp, Artificial Sequence
  Primer
  misc_feature (17)..(18): n is a, c, g, or t
  misc_feature (20)..(21): n is a, c, g, or t
  misc_feature (23)..(24): n is a, c, g, or t
gccatgagaattgttanntnnanncgggtttgtttcggacggca

SEQ ID NO: 309 - DNA, 45 bp, Artificial Sequence
  Primer
  misc_feature (16)..(17): n is a, c, g, or t
  misc_feature (19)..(20): n is a, c, g, or t
  misc_feature (22)..(23): n is a, c, g, or t
gaaacaaacccgtttnnanntnncaattctcatggcacacacgtc

SEQ ID NO: 310 - DNA, 44 bp, Artificial Sequence
  Primer
  misc_feature (17)..(18): n is a, c, g, or t
  misc_feature (20)..(21): n is a, c, g, or t
  misc_feature (23)..(24): n is a, c, g, or t
tgtgccatgagaattgnnanntnnaaacgggtttgtttcggacg

SEQ ID NO: 311 - DNA, 43 bp, Artificial Sequence
  Primer
  misc_feature (16)..(17): n is a, c, g, or t
  misc_feature (19)..(20): n is a, c, g, or t
  misc_feature (22)..(23): n is a, c, g, or t
acaaacccgtttcaanntnncnnttctcatggcacacacgtcg

SEQ ID NO: 312 - DNA, 46 bp, Artificial Sequence
  Primer
  misc_feature (17)..(18): n is a, c, g, or t
  misc_feature (20)..(21): n is a, c, g, or t
  misc_feature (23)..(24): n is a, c, g, or t
gtgtgtgccatgagaanngnnannttgaaacgggtttgtttcggac

SEQ ID NO: 313 - DNA, 43 bp, Artificial Sequence
  Primer
  misc_feature (16)..(17): n is a, c, g, or t
  misc_feature (19)..(20): n is a, c, g, or t
  misc_feature (22)..(23): n is a, c, g, or t
aacccgtttcaagatnncnntnntcatggcacacacgtcgcag

SEQ ID NO: 314 - DNA, 46 bp, Artificial Sequence
  Primer
  misc_feature (17)..(18): n is a, c, g, or t
  misc_feature (20)..(21): n is a, c, g, or t
  misc_feature (23)..(24): n is a, c, g, or t
gacgtgtgtgccatgannanngnnatcttgaaacgggtttgtttcg

SEQ ID NO: 315 - DNA, 43 bp, Artificial Sequence
  Primer
  misc_feature (16)..(17): n is a, c, g, or t
  misc_feature (19)..(20): n is a, c, g, or t
  misc_feature (22)..(23): n is a, c, g, or t
ccgtttcaagataacnntnntnntggcacacacgtcgcaggaa

SEQ ID NO: 316 - DNA, 47 bp, Artificial Sequence
  Primer
  misc_feature (17)..(18): n is a, c, g, or t
  misc_feature (20)..(21): n is a, c, g, or t
  misc_feature (23)..(24): n is a, c, g, or t
tgcgacgtgtgtgccannannanngttatcttgaaacgggtttgttt

SEQ ID NO: 317 - DNA, 44 bp, Artificial Sequence
  Primer
  misc_feature (16)..(17): n is a, c, g, or t
  misc_feature (19)..(20): n is a, c, g, or t
  misc_feature (22)..(23): n is a, c, g, or t
aattctcatggcacanncnncnnaggaacggttgcggcgttaaa

SEQ ID NO: 318 - DNA, 47 bp, Artificial Sequence
  Primer
  misc_feature (17)..(18): n is a, c, g, or t
  misc_feature (20)..(21): n is a, c, g, or t
  misc_feature (23)..(24): n is a, c, g, or t
cgccgcaaccgttcctnngnngnntgtgccatgagaattgttatctt

SEQ ID NO: 319 - DNA, 45 bp, Artificial Sequence
  Primer
  misc_feature (16)..(17): n is a, c, g, or t
  misc_feature (19)..(20): n is a, c, g, or t
  misc_feature (22)..(23): n is a, c, g, or t
tctcatggcacacacnncnnannaacggttgcggcgttaaacaat

SEQ ID NO: 320 - DNA, 46 bp, Artificial Sequence
  Primer
  misc_feature (17)..(18): n is a, c, g, or t
  misc_feature (20)..(21): n is a, c, g, or t
  misc_feature (23)..(24): n is a, c, g, or t
taacgccgcaaccgttnntnngnngtgtgtgccatgagaattgtta

SEQ ID NO: 321 - DNA, 47 bp, Artificial Sequence
  Primer
  misc_feature (16)..(17): n is a, c, g, or t
  misc_feature (19)..(20): n is a, c, g, or t
  misc_feature (22)..(23): n is a, c, g, or t
acacacgtcgcagganngnntnnggcgttaaacaattctattggcgt

SEQ ID NO: 322 - DNA, 44 bp, Artificial Sequence
  Primer
  misc_feature (17)..(18): n is a, c, g, or t
  misc_feature (20)..(21): n is a, c, g, or t
  misc_feature (23)..(24): n is a, c, g, or t
agaattgtttaacgccnnanncnntcctgcgacgtgtgtgccat

SEQ ID NO: 323 - DNA, 46 bp, Artificial Sequence
  Primer
  misc_feature (16)..(17): n is a, c, g, or t
  misc_feature (19)..(20): n is a, c, g, or t
  misc_feature (22)..(23): n is a, c, g, or t
gcaggaacggttgcgnngnnanncaattctattggcgtgcttggtg

SEQ ID NO: 324 - DNA, 44 bp, Artificial Sequence
  Primer
  misc_feature (17)..(18): n is a, c, g, or t
  misc_feature (20)..(21): n is a, c, g, or t
  misc_feature (23)..(24): n is a, c, g, or t
cacgccaatagaattgnntnncnncgcaaccgttcctgcgacgt

SEQ ID NO: 325 - DNA, 44 bp, Artificial Sequence
  Primer
  misc_feature (16)..(17): n is a, c, g, or t
  misc_feature (19)..(20): n is a, c, g, or t
  misc_feature (22)..(23): n is a, c, g, or t
acggttgcggcgttanncnntnntattggcgtgcttggtgtagc

SEQ ID NO: 326 - DNA, 44 bp, Artificial Sequence
  Primer
  misc_feature (17)..(18): n is a, c, g, or t
  misc_feature (20)..(21): n is a, c, g, or t
  misc_feature (23)..(24): n is a, c, g, or t
accaagcacgccaatannanngnntaacgccgcaaccgttcctg

SEQ ID NO: 327 - DNA, 44 bp, Artificial Sequence
  Primer
  misc_feature (16)..(17): n is a, c, g, or t
  misc_feature (19)..(20): n is a, c, g, or t
  misc_feature (22)..(23): n is a, c, g, or t
aacaattctattggcnngnntnntgtagccccgtctgcttcgct

SEQ ID NO: 328 - DNA, 50 bp, Artificial Sequence
  Primer
  misc_feature (17)..(18): n is a, c, g, or t
  misc_feature (20)..(21): n is a, c, g, or t
  misc_feature (23)..(24): n is a, c, g, or t
agcagacggggctacannanncnngccaatagaattgtttaacgccgcaa

SEQ ID NO: 329 - DNA, 43 bp, Artificial Sequence
  Primer
  misc_feature (16)..(17): n is a, c, g, or t
  misc_feature (19)..(20): n is a, c, g, or t
  misc_feature (22)..(23): n is a, c, g, or t
tctattggcgtgcttnntnnanncccgtctgcttcgctctacg

SEQ ID NO: 330 - DNA, 47 bp, Artificial Sequence
  Primer
  misc_feature (17)..(18): n is a, c, g, or t
  misc_feature (20)..(21): n is a, c, g, or t
  misc_feature (23)..(24): n is a, c, g, or t
gagcgaagcagacgggnntnnannaagcacgccaatagaattgttta

SEQ ID NO: 331 - DNA, 44 bp, Artificial Sequence
  Primer
  misc_feature (16)..(17): n is a, c, g, or t
  misc_feature (19)..(20): n is a, c, g, or t
  misc_feature (22)..(23): n is a, c, g, or t
attggcgtgcttggtnnanncnngtctgcttcgctctacgccgt

SEQ ID NO: 332 - DNA, 46 bp, Artificial Sequence
  Primer
  misc_feature (17)..(18): n is a, c, g, or t
  misc_feature (20)..(21): n is a, c, g, or t
  misc_feature (23)..(24): n is a, c, g, or t
gtagagcgaagcagacnngnntnnaccaagcacgccaatagaattg

SEQ ID NO: 333 - DNA, 45 bp, Artificial Sequence
  Primer
  misc_feature (17)..(18): n is a, c, g, or t
  misc_feature (20)..(21): n is a, c, g, or t
  misc_feature (23)..(24): n is a, c, g, or t
tggcgtgcttggtgtanncnngnntgcttcgctctacgccgttaa

SEQ ID NO: 334 - DNA, 45 bp, Artificial Sequence
  Primer
  misc_feature (17)..(18): n is a, c, g, or t
  misc_feature (20)..(21): n is a, c, g, or t
  misc_feature (23)..(24): n is a, c, g, or t
ggcgtagagcgaagcanncnngnntacaccaagcacgccaataga

SEQ ID NO: 335 - DNA, 45 bp, Artificial Sequence
  Primer
  misc_feature (16)..(17): n is a, c, g, or t
  misc_feature (19)..(20): n is a, c, g, or t
  misc_feature (22)..(23): n is a, c, g, or t
gtgcttggtgtagccnngnntnnttcgctctacgccgttaaagtt

SEQ ID NO: 336 - DNA, 44 bp, Artificial Sequence
  Primer
  misc_feature (17)..(18): n is a, c, g, or t
  misc_feature (20)..(21): n is a, c, g, or t
  misc_feature (23)..(24): n is a, c, g, or t
aacggcgtagagcgaannanncnnggctacaccaagcacgccaa

SEQ ID NO: 337 - DNA, 45 bp, Artificial Sequence
  Primer
  misc_feature (16)..(17): n is a, c, g, or t
  misc_feature (19)..(20): n is a, c, g, or t
  misc_feature (22)..(23): n is a, c, g, or t
cttggtgtagccccgnntnntnngctctacgccgttaaagttctt

SEQ ID NO: 338 - DNA, 48 bp, Artificial Sequence
  Primer
  misc_feature (17)..(18): n is a, c, g, or t
  misc_feature (20)..(21): n is a, c, g, or t
  misc_feature (23)..(24): n is a, c, g, or t
tttaacggcgtagagcnnannanncggggctacaccaagcacgccaat

SEQ ID NO: 339 - DNA, 46 bp, Artificial Sequence
  Primer
  misc_feature (16)..(17): n is a, c, g, or t
  misc_feature (19)..(20): n is a, c, g, or t
  misc_feature (22)..(23): n is a, c, g, or t
ggtgtagccccgtctnntnngnnctacgccgttaaagttcttgcag

SEQ ID NO: 340 - DNA, 44 bp, Artificial Sequence
  Primer
  misc_feature (17)..(18): n is a, c, g, or t
  misc_feature (20)..(21): n is a, c, g, or t
  misc_feature (23)..(24): n is a, c, g, or t
aactttaacggcgtagnncnnannagacggggctacaccaagca

SEQ ID NO: 341 - DNA, 45 bp, Artificial Sequence
  Primer
  misc_feature (16)..(17): n is a, c, g, or t
  misc_feature (19)..(20): n is a, c, g, or t
  misc_feature (22)..(23): n is a, c, g, or t
gtagccccgtctgctnngnncnncgccgttaaagttcttgcagca

SEQ ID NO: 342 - DNA, 44 bp, Artificial Sequence
  Primer
  misc_feature (17)..(18): n is a, c, g, or t
  misc_feature (20)..(21): n is a, c, g, or t
  misc_feature (23)..(24): n is a, c, g, or t
aagaactttaacggcgnngnncnnagcagacggggctacaccaa

SEQ ID NO: 343 - DNA, 45 bp, Artificial Sequence
  Primer
  misc_feature (16)..(17): n is a, c, g, or t
  misc_feature (19)..(20): n is a, c, g, or t
  misc_feature (22)..(23): n is a, c, g, or t
gccccgtctgcttcgnncnncnncgttaaagttcttgcagcagac

SEQ ID NO: 344 - DNA, 44 bp, Artificial Sequence
  Primer
  misc_feature (17)..(18): n is a, c, g, or t
  misc_feature (20)..(21): n is a, c, g, or t
  misc_feature (23)..(24): n is a, c, g, or t
tgcaagaactttaacgnngnngnncgaagcagacggggctacac

SEQ ID NO: 345 - DNA, 45 bp, Artificial Sequence
  Primer
  misc_feature (16)..(17): n is a, c, g, or t
  misc_feature (19)..(20): n is a, c, g, or t
  misc_feature (22)..(23): n is a, c, g, or t
ccgtctgcttcgctcnncnncnntaaagttcttgcagcagacgga

SEQ ID NO: 346 - DNA, 43 bp, Artificial Sequence
  Primer
  misc_feature (17)..(18): n is a, c, g, or t
  misc_feature (20)..(21): n is a, c, g, or t
  misc_feature (23)..(24): n is a, c, g, or t
tgctgcaagaactttanngnngnngagcgaagcagacggggct

SEQ ID NO: 347 - DNA, 44 bp, Artificial Sequence
  Primer
  misc_feature (16)..(17): n is a, c, g, or t
  misc_feature (19)..(20): n is a, c, g, or t
  misc_feature (22)..(23): n is a, c, g, or t
tctgcttcgctctacnncnntnnagttcttgcagcagacggatc

SEQ ID NO: 348 - DNA, 47 bp, Artificial Sequence
  Primer
  misc_feature (17)..(18): n is a, c, g, or t
  misc_feature (20)..(21): n is a, c, g, or t
  misc_feature (23)..(24): n is a, c, g, or t
gtctgctgcaagaactnnanngnngtagagcgaagcagacggggcta

SEQ ID NO: 349 - DNA, 43 bp, Artificial Sequence
  Primer
  misc_feature (16)..(17): n is a, c, g, or t
  misc_feature (19)..(20): n is a, c, g, or t
  misc_feature (22)..(23): n is a, c, g, or t
gcttcgctctacgccnntnnanntcttgcagcagacggatcag

SEQ ID NO: 350 - DNA, 44 bp, Artificial Sequence
  Primer
  misc_feature (17)..(18): n is a, c, g, or t
  misc_feature (20)..(21): n is a, c, g, or t
  misc_feature (23)..(24): n is a, c, g, or t
tccgtctgctgcaaganntnnannggcgtagagcgaagcagacg

SEQ ID NO: 351 - DNA, 44 bp, Artificial Sequence
  Primer
  misc_feature (16)..(17): n is a, c, g, or t
  misc_feature (19)..(20): n is a, c, g, or t
  misc_feature (22)..(23): n is a, c, g, or t
tcgctctacgccgttnnanntnntgcagcagacggatcaggcca

SEQ ID NO: 352 - DNA, 44 bp, Artificial Sequence
  Primer
  misc_feature (17)..(18): n is a, c, g, or t
  misc_feature (20)..(21): n is a, c, g, or t
  misc_feature (23)..(24): n is a, c, g, or t
tgatccgtctgctgcannanntnnaacggcgtagagcgaagcag

SEQ ID NO: 353 - DNA, 44 bp, Artificial Sequence
  Primer
  misc_feature (16)..(17): n is a, c, g, or t
  misc_feature (19)..(20): n is a, c, g, or t
  misc_feature (22)..(23): n is a, c, g, or t
ctctacgccgttaaanntnntnnagcagacggatcaggccaata

SEQ ID NO: 354 - DNA, 44 bp, Artificial Sequence
  Primer
  misc_feature (17)..(18): n is a, c, g, or t
  misc_feature (20)..(21): n is a, c, g, or t
  misc_feature (23)..(24): n is a, c, g, or t
gcctgatccgtctgctnnannanntttaacggcgtagagcgaag

SEQ ID NO: 355 - DNA, 44 bp, Artificial Sequence
  Primer
  misc_feature (16)..(17): n is a, c, g, or t
  misc_feature (19)..(20): n is a, c, g, or t
  misc_feature (22)..(23): n is a, c, g, or t
tacgccgttaaagttnntnnannagacggatcaggccaatactc

SEQ ID NO: 356 - DNA, 45 bp, Artificial Sequence
  Primer
  misc_feature (17)..(18): n is a, c, g, or t
  misc_feature (20)..(21): n is a, c, g, or t
  misc_feature (23)..(24): n is a, c, g, or t
ttggcctgatccgtctnntnnannaactttaacggcgtagagcga

SEQ ID NO: 357 - DNA, 44 bp, Artificial Sequence
  Primer
  misc_feature (16)..(17): n is a, c, g, or t
  misc_feature (19)..(20): n is a, c, g, or t
  misc_feature (22)..(23): n is a, c, g, or t
gccgttaaagttcttnnannanncggatcaggccaatactcatg

SEQ ID NO: 358 - DNA, 45 bp, Artificial Sequence
  Primer
  misc_feature (17)..(18): n is a, c, g, or t
  misc_feature (20)..(21): n is a, c, g, or t
  misc_feature (23)..(24): n is a, c, g, or t
gtattggcctgatccgnntnntnnaagaactttaacggcgtagag

SEQ ID NO: 359 - DNA, 46 bp, Artificial Sequence
  Primer
  misc_feature (16)..(17): n is a, c, g, or t
  misc_feature (19)..(20): n is a, c, g, or t
  misc_feature (22)..(23): n is a, c, g, or t
gttaaagttcttgcannanncnnatcaggccaatactcatggatta

SEQ ID NO: 360 - DNA, 46 bp, Artificial Sequence
  Primer
  misc_feature (17)..(18): n is a, c, g, or t
  misc_feature (20)..(21): n is a, c, g, or t
  misc_feature (23)..(24): n is a, c, g, or t
tgagtattggcctgatnngnntnntgcaagaactttaacggcgtag

SEQ ID NO: 361 - DNA, 45 bp, Artificial Sequence
  Primer
  misc_feature (16)..(17): n is a, c, g, or t
  misc_feature (19)..(20): n is a, c, g, or t
  misc_feature (22)..(23): n is a, c, g, or t
aaagttcttgcagcanncnnannaggccaatactcatggattatc

SEQ ID NO: 362 - DNA, 48 bp, Artificial Sequence
  Primer
  misc_feature (17)..(18): n is a, c, g, or t
  misc_feature (20)..(21): n is a, c, g, or t
  misc_feature (23)..(24): n is a, c, g, or t
ccatgagtattggcctnntnngnntgctgcaagaactttaacggcgta

SEQ ID NO: 363 - DNA, 45 bp, Artificial Sequence
  Primer
  misc_feature (16)..(17): n is a, c, g, or t
  misc_feature (19)..(20): n is a, c, g, or t
  misc_feature (22)..(23): n is a, c, g, or t
gttcttgcagcagacnnannannccaatactcatggattatcaac

SEQ ID NO: 364 - DNA, 46 bp, Artificial Sequence
  Primer
  misc_feature (17)..(18): n is a, c, g, or t
  misc_feature (20)..(21): n is a, c, g, or t
  misc_feature (23)..(24): n is a, c, g, or t
aatccatgagtattggnntnntnngtctgctgcaagaactttaacg

SEQ ID NO: 365 - DNA, 46 bp, Artificial Sequence
  Primer
  misc_feature (16)..(17): n is a, c, g, or t
  misc_feature (19)..(20): n is a, c, g, or t
  misc_feature (22)..(23): n is a, c, g, or t
cttgcagcagacggannanncnnatactcatggattatcaacggca

SEQ ID NO: 366 - DNA, 45 bp, Artificial Sequence
  Primer
  misc_feature (17)..(18): n is a, c, g, or t
  misc_feature (20)..(21): n is a, c, g, or t
  misc_feature (23)..(24): n is a, c, g, or t
gataatccatgagtatnngnntnntccgtctgctgcaagaacttt

SEQ ID NO: 367 - DNA, 45 bp, Artificial Sequence
  Primer
  misc_feature (16)..(17): n is a, c, g, or t
  misc_feature (19)..(20): n is a, c, g, or t
  misc_feature (22)..(23): n is a, c, g, or t
gcagcagacggatcanncnnannctcatggattatcaacggcatc

SEQ ID NO: 368 - DNA, 44 bp, Artificial Sequence
  Primer
  misc_feature (16)..(17): n is a, c, g, or t
  misc_feature (19)..(20): n is a, c, g, or t
  misc_feature (22)..(23): n is a, c, g, or t
ttgataatccatgagnntnngnntgatccgtctgctgcaagaac

SEQ ID NO: 369 - DNA, 46 bp, Artificial Sequence
  Primer
  misc_feature (16)..(17): n is a, c, g, or t
  misc_feature (19)..(20): n is a, c, g, or t
  misc_feature (22)..(23): n is a, c, g, or t
gcagacggatcaggcnnanncnnatggattatcaacggcatcgaat

SEQ ID NO: 370 - DNA, 44 bp, Artificial Sequence
  Primer
  misc_feature (17)..(18): n is a, c, g, or t
  misc_feature (20)..(21): n is a, c, g, or t
  misc_feature (23)..(24): n is a, c, g, or t
gccgttgataatccatnngnntnngcctgatccgtctgctgcaa

SEQ ID NO: 371 - DNA, 45 bp, Artificial Sequence
  Primer
  misc_feature (16)..(17): n is a, c, g, or t
  misc_feature (19)..(20): n is a, c, g, or t
  misc_feature (22)..(23): n is a, c, g, or t
gacggatcaggccaanncnnanngattatcaacggcatcgaatgg

SEQ ID NO: 372 - DNA, 44 bp, Artificial Sequence
  Primer
  misc_feature (17)..(18): n is a, c, g, or t
  misc_feature (20)..(21): n is a, c, g, or t
  misc_feature (23)..(24): n is a, c, g, or t
gatgccgttgataatcnntnngnnttggcctgatccgtctgctg

SEQ ID NO: 373 - DNA, 47 bp, Artificial Sequence
  Primer
  misc_feature (16)..(17): n is a, c, g, or t
  misc_feature (19)..(20): n is a, c, g, or t
  misc_feature (22)..(23): n is a, c, g, or t
ggatcaggccaatacnnanngnntatcaacggcatcgaatgggccat

SEQ ID NO: 374 - DNA, 44 bp, Artificial Sequence
  Primer
  misc_feature (17)..(18): n is a, c, g, or t
  misc_feature (20)..(21): n is a, c, g, or t
  misc_feature (23)..(24): n is a, c, g, or t
ttcgatgccgttgatanncnntnngtattggcctgatccgtctg

SEQ ID NO: 375 - DNA, 44 bp, Artificial Sequence
  Primer
  misc_feature (16)..(17): n is a, c, g, or t
  misc_feature (19)..(20): n is a, c, g, or t
  misc_feature (22)..(23): n is a, c, g, or t
tcaggccaatactcanngnntnncaacggcatcgaatgggccat

SEQ ID NO: 376 - DNA, 45 bp, Artificial Sequence
  Primer
  misc_feature (17)..(18): n is a, c, g, or t
  misc_feature (20)..(21): n is a, c, g, or t
  misc_feature (23)..(24): n is a, c, g, or t
ccattcgatgccgttgnnanncnntgagtattggcctgatccgtc

SEQ ID NO: 377 - DNA, 48 bp, Artificial Sequence
  Primer
  misc_feature (16)..(17): n is a, c, g, or t
  misc_feature (19)..(20): n is a, c, g, or t
  misc_feature (22)..(23): n is a, c, g, or t
ggccaatactcatggnntnncnncggcatcgaatgggccatcgcgaat

SEQ ID NO: 378 - DNA, 45 bp, Artificial Sequence
  Primer
  misc_feature (17)..(18): n is a, c, g, or t
  misc_feature (20)..(21): n is a, c, g, or t
  misc_feature (23)..(24): n is a, c, g, or t
ggcccattcgatgccgnngnnannccatgagtattggcctgatcc

SEQ ID NO: 379 - DNA, 44 bp, Artificial Sequence
  Primer
  misc_feature (16)..(17): n is a, c, g, or t
  misc_feature (19)..(20): n is a, c, g, or t
  misc_feature (22)..(23): n is a, c, g, or t
caatactcatggattnncnncnncatcgaatgggccatcgcgaa

SEQ ID NO: 380 - DNA, 46 bp, Artificial Sequence
  Primer
  misc_feature (17)..(18): n is a, c, g, or t
  misc_feature (20)..(21): n is a, c, g, or t
  misc_feature (23)..(24): n is a, c, g, or t
gatggcccattcgatgnngnngnnaatccatgagtattggcctgat

SEQ ID NO: 381 - DNA, 44 bp, Artificial Sequence
  Primer
  misc_feature (16)..(17): n is a, c, g, or t
  misc_feature (19)..(20): n is a, c, g, or t
  misc_feature (22)..(23): n is a, c, g, or t
tactcatggattatcnncnncnncgaatgggccatcgcgaataa

SEQ ID NO: 382 - DNA, 46 bp, Artificial Sequence
  Primer
  misc_feature (17)..(18): n is a, c, g, or t
  misc_feature (20)..(21): n is a, c, g, or t
  misc_feature (23)..(24): n is a, c, g, or t
cgcgatggcccattcgnngnngnngataatccatgagtattggcct

SEQ ID NO: 383 - DNA, 45 bp, Artificial Sequence
  Primer
  misc_feature (16)..(17): n is a, c, g, or t
  misc_feature (19)..(20): n is a, c, g, or t
  misc_feature (22)..(23): n is a, c, g, or t
tcatggattatcaacnncnncnnatgggccatcgcgaataacatg

SEQ ID NO: 384 - DNA, 46 bp, Artificial Sequence
  Primer
  misc_feature (17)..(18): n is a, c, g, or t
  misc_feature (20)..(21): n is a, c, g, or t
  misc_feature (23)..(24): n is a, c, g, or t
attcgcgatggcccatnngnngnngttgataatccatgagtattgg

SEQ ID NO: 385 - DNA, 44 bp, Artificial Sequence
  Primer
  misc_feature (16)..(17): n is a, c, g, or t
  misc_feature (19)..(20): n is a, c, g, or t
  misc_feature (22)..(23): n is a, c, g, or t
tggattatcaacggcnncnnannggccatcgcgaataacatgga

SEQ ID NO: 386 - DNA, 46 bp, Artificial Sequence
  Primer
  misc_feature (17)..(18): n is a, c, g, or t
  misc_feature (20)..(21): n is a, c, g, or t
  misc_feature (23)..(24): n is a, c, g, or t
gttattcgcgatggccnntnngnngccgttgataatccatgagtat

SEQ ID NO: 387 - DNA, 46 bp, Artificial Sequence
  Primer
  misc_feature (16)..(17): n is a, c, g, or t
  misc_feature (19)..(20): n is a, c, g, or t
  misc_feature (22)..(23): n is a, c, g, or t
attatcaacggcatcnnanngnncatcgcgaataacatggatgtaa

SEQ ID NO: 388 - DNA, 46 bp, Artificial Sequence
  Primer
  misc_feature (17)..(18): n is a, c, g, or t
  misc_feature (20)..(21): n is a, c, g, or t
  misc_feature (23)..(24): n is a, c, g, or t
catgttattcgcgatgnncnntnngatgccgttgataatccatgag

SEQ ID NO: 389 - DNA, 47 bp, Artificial Sequence
  Primer
  misc_feature (16)..(17): n is a, c, g, or t
  misc_feature (19)..(20): n is a, c, g, or t
  misc_feature (22)..(23): n is a, c, g, or t
atcaacggcatcgaanngnncnncgcgaataacatggatgtaatcaa

SEQ ID NO: 390 - DNA, 46 bp, Artificial Sequence
  Primer
  misc_feature (17)..(18): n is a, c, g, or t
  misc_feature (20)..(21): n is a, c, g, or t
  misc_feature (23)..(24): n is a, c, g, or t
atccatgttattcgcgnngnncnnttcgatgccgttgataatccat

SEQ ID NO: 391 - DNA, 47 bp, Artificial Sequence
  Primer
  misc_feature (16)..(17): n is a, c, g, or t
  misc_feature (19)..(20): n is a, c, g, or t
  misc_feature (22)..(23): n is a, c, g, or t
aacggcatcgaatggnncnncnngaataacatggatgtaatcaacat

SEQ ID NO: 392 - DNA, 47 bp, Artificial Sequence; identical to SEQ ID NO: 391
  Primer
  misc_feature (16)..(17): n is a, c, g, or t
  misc_feature (19)..(20): n is a, c, g, or t
  misc_feature (22)..(23): n is a, c, g, or t

SEQ ID NO: 393 - DNA, 47 bp, Artificial Sequence
  Primer
  misc_feature (16)..(17): n is a, c, g, or t
  misc_feature (19)..(20): n is a, c, g, or t
  misc_feature (22)..(23): n is a, c, g, or t
ggcatcgaatgggccnncnngnntaacatggatgtaatcaacatgag

SEQ ID NO: 394 - DNA, 44 bp, Artificial Sequence
  Primer
  misc_feature (17)..(18): n is a, c, g, or t
  misc_feature (20)..(21): n is a, c, g, or t
  misc_feature (23)..(24): n is a, c, g, or t
gattacatccatgttanncnngnnggcccattcgatgccgttga

SEQ ID NO: 395 - DNA, 47 bp, Artificial Sequence
  Primer
  misc_feature (16)..(17): n is a, c, g, or t
  misc_feature (19)..(20): n is a, c, g, or t
  misc_feature (22)..(23): n is a, c, g, or t
atcgaatgggccatcnngnntnncatggatgtaatcaacatgagcct

SEQ ID NO: 396 - DNA, 44 bp, Artificial Sequence
  Primer
  misc_feature (17)..(18): n is a, c, g, or t
  misc_feature (20)..(21): n is a, c, g, or t
  misc_feature (23)..(24): n is a, c, g, or t
gttgattacatccatgnnanncnngatggcccattcgatgccgt

SEQ ID NO: 397 - DNA, 45 bp, Artificial Sequence
  Primer
  misc_feature (16)..(17): n is a, c, g, or t
  misc_feature (19)..(20): n is a, c, g, or t
  misc_feature (22)..(23): n is a, c, g, or t
gaatgggccatcgcgnntnncnnggatgtaatcaacatgagcctg

SEQ ID NO: 398 - DNA, 44 bp, Artificial Sequence
  Primer
  misc_feature (17)..(18): n is a, c, g, or t
  misc_feature (20)..(21): n is a, c, g, or t
  misc_feature (23)..(24): n is a, c, g, or t
catgttgattacatccnngnnanncgcgatggcccattcgatgc

SEQ ID NO: 399 - DNA, 45 bp, Artificial Sequence
  Primer
  misc_feature (16)..(17): n is a, c, g, or t
  misc_feature (19)..(20): n is a, c, g, or t
  misc_feature (22)..(23): n is a, c, g, or t
tgggccatcgcgaatnncnngnntgtaatcaacatgagcctggga

SEQ ID NO: 400 - DNA, 44 bp, Artificial Sequence
  Primer
  misc_feature (17)..(18): n is a, c, g, or t
  misc_feature (20)..(21): n is a, c, g, or t
  misc_feature (23)..(24): n is a, c, g, or t
gctcatgttgattacanncnngnnattcgcgatggcccattcga

SEQ ID NO: 401 - DNA, 45 bp, Artificial Sequence
  Primer
  misc_feature (16)..(17): n is a, c, g, or t
  misc_feature (19)..(20): n is a, c, g, or t
  misc_feature (22)..(23): n is a, c, g, or t
gccatcgcgaataacnngnntnnaatcaacatgagcctgggagca

SEQ ID NO: 402 - DNA, 45 bp, Artificial Sequence
  Primer
  misc_feature (17)..(18): n is a, c, g, or t
  misc_feature (20)..(21): n is a, c, g, or t
  misc_feature (23)..(24): n is a, c, g, or t
caggctcatgttgattnnanncnngttattcgcgatggcccattc

SEQ ID NO: 403 - DNA, 43 bp, Artificial Sequence
  Primer
  misc_feature (16)..(17): n is a, c, g, or t
  misc_feature (19)..(20): n is a, c, g, or t
  misc_feature (22)..(23): n is a, c, g, or t
atcgcgaataacatgnntnnanncaacatgagcctgggagcac

SEQ ID NO: 404 - DNA, 46 bp, Artificial Sequence
  Primer
  misc_feature (17)..(18): n is a, c, g, or t
  misc_feature (20)..(21): n is a, c, g, or t
  misc_feature (23)..(24): n is a, c, g, or t
tcccaggctcatgttgnntnnanncatgttattcgcgatggcccat

SEQ ID NO: 405 - DNA, 44 bp, Artificial Sequence
  Primer
  misc_feature (16)..(17): n is a, c, g, or t
  misc_feature (19)..(20): n is a, c, g, or t
  misc_feature (22)..(23): n is a, c, g, or t
gcgaataacatggatnnanncnncatgagcctgggagcaccaag

SEQ ID NO: 406 - DNA, 50 bp, Artificial Sequence
  Primer
  misc_feature (17)..(18): n is a, c, g, or t
  misc_feature (20)..(21): n is a, c, g, or t
  misc_feature (23)..(24): n is a, c, g, or t
tgctcccaggctcatgnngnntnnatccatgttattcgcgatggcccatt

SEQ ID NO: 407 - DNA, 46 bp, Artificial Sequence
  Primer
  misc_feature (16)..(17): n is a, c, g, or t
  misc_feature (19)..(20): n is a, c, g, or t
  misc_feature (22)..(23): n is a, c, g, or t
aataacatggatgtanncnncnngagcctgggagcaccaagcggca

SEQ ID NO: 408 - DNA, 46 bp, Artificial Sequence
  Primer
  misc_feature (17)..(18): n is a, c, g, or t
  misc_feature (20)..(21): n is a, c, g, or t
  misc_feature (23)..(24): n is a, c, g, or t
tggtgctcccaggctcnngnngnntacatccatgttattcgcgatg

SEQ ID NO: 409 - DNA, 43 bp, Artificial Sequence
  Primer
  misc_feature (16)..(17): n is a, c, g, or t
  misc_feature (19)..(20): n is a, c, g, or t
  misc_feature (22)..(23): n is a, c, g, or t
aacatggatgtaatcnncnngnncctgggagcaccaagcggca

SEQ ID NO: 410 - DNA, 47 bp, Artificial Sequence
  Primer
  misc_feature (17)..(18): n is a, c, g, or t
  misc_feature (20)..(21): n is a, c, g, or t
  misc_feature (23)..(24): n is a, c, g, or t
gcttggtgctcccaggnncnngnngattacatccatgttattcgcga

SEQ ID NO: 411 - DNA, 43 bp, Artificial Sequence
  Primer
  misc_feature (16)..(17): n is a, c, g, or t
  misc_feature (19)..(20): n is a, c, g, or t
  misc_feature (22)..(23): n is a, c, g, or t
atggatgtaatcaacnngnncnngggagcaccaagcggcagtg

SEQ ID NO: 412 - DNA, 47 bp, Artificial Sequence
  Primer
  misc_feature (17)..(18): n is a, c, g, or t
  misc_feature (20)..(21): n is a, c, g, or t
  misc_feature (23)..(24): n is a, c, g, or t
gccgcttggtgctcccnngnncnngttgattacatccatgttattcg

SEQ ID NO: 413 - DNA, 45 bp, Artificial Sequence
  Primer
  misc_feature (16)..(17): n is a, c, g, or t
  misc_feature (19)..(20): n is a, c, g, or t
  misc_feature (22)..(23): n is a, c, g, or t
gatgtaatcaacatgnncnngnnagcaccaagcggcagtgcggca

SEQ ID NO: 414 - DNA, 48 bp, Artificial Sequence
  Primer
  misc_feature (17)..(18): n is a, c, g, or t
  misc_feature (20)..(21): n is a, c, g, or t
  misc_feature (23)..(24): n is a, c, g, or t
actgccgcttggtgctnncnngnncatgttgattacatccatgttatt

SEQ ID NO: 415 - DNA, 44 bp, Artificial Sequence
  Primer
  misc_feature (16)..(17): n is a, c, g, or t
  misc_feature (19)..(20): n is a, c, g, or t
  misc_feature (22)..(23): n is a, c, g, or t
gtaatcaacatgagcnngnnannaccaagcggcagtgcggcact

SEQ ID NO: 416 - DNA, 46 bp, Artificial Sequence
  Primer
  misc_feature (17)..(18): n is a, c, g, or t
  misc_feature (20)..(21): n is a, c, g, or t
  misc_feature (23)..(24): n is a, c, g, or t
cgcactgccgcttggtnntnncnngctcatgttgattacatccatg

SEQ ID NO: 417 - DNA, 45 bp, Artificial Sequence
  Primer
  misc_feature (16)..(17): n is a, c, g, or t
  misc_feature (19)..(20): n is a, c, g, or t
  misc_feature (22)..(23): n is a, c, g, or t
atgagcctgggagcannanncnncagtgcggcacttaaagcagca

SEQ ID NO: 418 - DNA, 45 bp, Artificial Sequence
  Primer
  misc_feature (17)..(18): n is a, c, g, or t
  misc_feature (20)..(21): n is a, c, g, or t
  misc_feature (23)..(24): n is a, c, g, or t
tttaagtgccgcactgnngnntnntgctcccaggctcatgttgat

SEQ ID NO: 419 - DNA, 46 bp, Artificial Sequence
  Primer
  misc_feature (16)..(17): n is a, c, g, or t
  misc_feature (19)..(20): n is a, c, g, or t
  misc_feature (22)..(23): n is a, c, g, or t
ggagcaccaagcggcnntnngnnacttaaagcagcagttgataaag

SEQ ID NO: 420 - DNA, 45 bp, Artificial Sequence
  Primer
  misc_feature (17)..(18): n is a, c, g, or t
  misc_feature (20)..(21): n is a, c, g, or t
  misc_feature (23)..(24): n is a, c, g, or t
aactgctgctttaagtnncnnanngccgcttggtgctcccaggct

SEQ ID NO: 421 - DNA, 46 bp, Artificial Sequence
  Primer
  misc_feature (16)..(17): n is a, c, g, or t
  misc_feature (19)..(20): n is a, c, g, or t
  misc_feature (22)..(23): n is a, c, g, or t
gcaccaagcggcagtnngnnanntaaagcagcagttgataaagctg

SEQ ID NO: 422 - DNA, 44 bp, Artificial Sequence
  Primer
  misc_feature (17)..(18): n is a, c, g, or t
  misc_feature (20)..(21): n is a, c, g, or t
  misc_feature (23)..(24): n is a, c, g, or t
atcaactgctgctttanntnncnnactgccgcttggtgctccca

SEQ ID NO: 423 - DNA, 46 bp, Artificial Sequence
  Primer
  misc_feature (16)..(17): n is a, c, g, or t
  misc_feature (19)..(20): n is a, c, g, or t
  misc_feature (22)..(23): n is a, c, g, or t
ccaagcggcagtgcgnnanntnnagcagcagttgataaagctgttg

SEQ ID NO: 424 - DNA, 44 bp, Artificial Sequence
  Primer
  misc_feature (17)..(18): n is a, c, g, or t
  misc_feature (20)..(21): n is a, c, g, or t
  misc_feature (23)..(24): n is a, c, g, or t
tttatcaactgctgctnnanntnncgcactgccgcttggtgctc

SEQ ID NO: 425 - DNA, 46 bp, Artificial Sequence
  Primer
  misc_feature (16)..(17): n is a, c, g, or t
  misc_feature (19)..(20): n is a, c, g, or t
  misc_feature (22)..(23): n is a, c, g, or t
agcggcagtgcggcanntnnannagcagttgataaagctgttgcat

SEQ ID NO: 426 - DNA, 44 bp, Artificial Sequence
  Primer
  misc_feature (17)..(18): n is a, c, g, or t
  misc_feature (20)..(21): n is a, c, g, or t
  misc_feature (23)..(24): n is a, c, g, or t
agctttatcaactgctnntnnanntgccgcactgccgcttggtg

SEQ ID NO: 427 - DNA, 46 bp, Artificial Sequence
  Primer
  misc_feature (16)..(17): n is a, c, g, or t
  misc_feature (19)..(20): n is a, c, g, or t
  misc_feature (22)..(23): n is a, c, g, or t
ggcagtgcggcacttnnannannagttgataaagctgttgcatctg

SEQ ID NO: 428 - DNA, 44 bp, Artificial Sequence
  Primer
  misc_feature (17)..(18): n is a, c, g, or t
  misc_feature (20)..(21): n is a, c, g, or t
  misc_feature (23)..(24): n is a, c, g, or t
aacagctttatcaactnntnntnnaagtgccgcactgccgcttg

SEQ ID NO: 429 - DNA, 46 bp, Artificial Sequence
  Primer
  misc_feature (16)..(17): n is a, c, g, or t
  misc_feature (19)..(20): n is a, c, g, or t
  misc_feature (22)..(23): n is a, c, g, or t
agtgcggcacttaaannannanntgataaagctgttgcatctggtg

SEQ ID NO: 430 - DNA, 46 bp, Artificial Sequence
  Primer
  misc_feature (17)..(18): n is a, c, g, or t
  misc_feature (20)..(21): n is a, c, g, or t
  misc_feature (23)..(24): n is a, c, g, or t
tgcaacagctttatcanntnntnntttaagtgccgcactgccgctt

SEQ ID NO: 431 - DNA, 45 bp, Artificial Sequence
  Primer
  misc_feature (16)..(17): n is a, c, g, or t
  misc_feature (19)..(20): n is a, c, g, or t
  misc_feature (22)..(23): n is a, c, g, or t
gcggcacttaaagcannanntnntaaagctgttgcatctggtgtc

SEQ ID NO: 432 - DNA, 44 bp, Artificial Sequence
  Primer
  misc_feature (17)..(18): n is a, c, g, or t
  misc_feature (20)..(21): n is a, c, g, or t
  misc_feature (23)..(24): n is a, c, g, or t
agatgcaacagctttannanntnntgctttaagtgccgcactgc

SEQ ID NO: 433 - DNA, 44 bp, Artificial Sequence
  Primer
  misc_feature (16)..(17): n is a, c, g, or t
  misc_feature (19)..(20): n is a, c, g, or t
  misc_feature (22)..(23): n is a, c, g, or t
gcacttaaagcagcanntnntnnagctgttgcatctggtgtcgt

SEQ ID NO: 434 - DNA, 44 bp, Artificial Sequence
  Primer
  misc_feature (17)..(18): n is a, c, g, or t
  misc_feature (20)..(21): n is a, c, g, or t
  misc_feature (23)..(24): n is a, c, g, or t
accagatgcaacagctnnannanntgctgctttaagtgccgcac

SEQ ID NO: 435 - DNA, 44 bp, Artificial Sequence
  Primer
  misc_feature (16)..(17): n is a, c, g, or t
  misc_feature (19)..(20): n is a, c, g, or t
  misc_feature (22)..(23): n is a, c, g, or t
cttaaagcagcagttnntnnanntgttgcatctggtgtcgtcgt

SEQ ID NO: 436 - DNA, 46 bp, Artificial Sequence
  Primer
  misc_feature (17)..(18): n is a, c, g, or t
  misc_feature (20)..(21): n is a, c, g, or t
  misc_feature (23)..(24): n is a, c, g, or t
gacaccagatgcaacanntnnannaactgctgctttaagtgccgca

SEQ ID NO: 437 - DNA, 44 bp, Artificial Sequence
  Primer
  misc_feature (16)..(17): n is a, c, g, or t
  misc_feature (19)..(20): n is a, c, g, or t
  misc_feature (22)..(23): n is a, c, g, or t
aaagcagcagttgatnnanntnntgcatctggtgtcgtcgtagt

SEQ ID NO: 438 - DNA, 45 bp, Artificial Sequence
  Primer
  misc_feature (17)..(18): n is a, c, g, or t
  misc_feature (20)..(21): n is a, c, g, or t
  misc_feature (23)..(24): n is a, c, g, or t
gacgacaccagatgcannanntnnatcaactgctgctttaagtgc

SEQ ID NO: 439 - DNA, 44 bp, Artificial Sequence
  Primer
  misc_feature (16)..(17): n is a, c, g, or t
  misc_feature (19)..(20): n is a, c, g, or t
  misc_feature (22)..(23): n is a, c, g, or t
gcagcagttgataaanntnntnnatctggtgtcgtcgtagtagc

SEQ ID NO: 440 - DNA, 47 bp, Artificial Sequence
  Primer
  misc_feature (17)..(18): n is a, c, g, or t
  misc_feature (20)..(21): n is a, c, g, or t
  misc_feature (23)..(24): n is a, c, g, or t
tacgacgacaccagatnnannanntttatcaactgctgctttaagtg

SEQ ID NO: 441 - DNA, 45 bp, Artificial Sequence
  Primer
  misc_feature (16)..(17): n is a, c, g, or t
  misc_feature (19)..(20): n is a, c, g, or t
  misc_feature (22)..(23): n is a, c, g, or t
gcagttgataaagctnntnnanntggtgtcgtcgtagtagcggca

SEQ ID NO: 442 - DNA, 47 bp, Artificial Sequence
  Primer
  misc_feature (17)..(18): n is a, c, g, or t
  misc_feature (20)..(21): n is a, c, g, or t
  misc_feature (23)..(24): n is a, c, g, or t
tactacgacgacaccanntnnannagctttatcaactgctgctttaa

SEQ ID NO: 443 - DNA, 45 bp, Artificial Sequence
  Primer
  misc_feature (16)..(17): n is a, c, g, or t
  misc_feature (19)..(20): n is a, c, g, or t
  misc_feature (22)..(23): n is a, c, g, or t
gttgataaagctgttnnanntnntgtcgtcgtagtagcggcagct

SEQ ID NO: 444 - DNA, 46 bp, Artificial Sequence
  Primer
  misc_feature (17)..(18): n is a, c, g, or t
  misc_feature (20)..(21): n is a, c, g, or t
  misc_feature (23)..(24): n is a, c, g, or t
cgctactacgacgacannanntnnaacagctttatcaactgctgct

SEQ ID NO: 445 - DNA, 43 bp, Artificial Sequence
  Primer
  misc_feature (16)..(17): n is a, c, g, or t
  misc_feature (19)..(20): n is a, c, g, or t
  misc_feature (22)..(23): n is a, c, g, or t
gataaagctgttgcanntnntnncgtcgtagtagcggcagctg

SEQ ID NO: 446 - DNA, 46 bp, Artificial Sequence
  Primer
  misc_feature (17)..(18): n is a, c, g, or t
  misc_feature (20)..(21): n is a, c, g, or t
  misc_feature (23)..(24): n is a, c, g, or t
tgccgctactacgacgnnannanntgcaacagctttatcaactgct

SEQ ID NO: 447 - DNA, 44 bp, Artificial Sequence
  Primer
  misc_feature (16)..(17): n is a, c, g, or t
  misc_feature (19)..(20): n is a, c, g, or t
  misc_feature (22)..(23): n is a, c, g, or t
aaagctgttgcatctnntnncnncgtagtagcggcagctgggaa

SEQ ID NO: 448 - DNA, 47 bp, Artificial Sequence
  Primer
  misc_feature (17)..(18): n is a, c, g, or t
  misc_feature (20)..(21): n is a, c, g, or t
  misc_feature (23)..(24): n is a, c, g, or t
agctgccgctactacgnngnnannagatgcaacagctttatcaactg

SEQ ID NO: 449 - DNA, 44 bp, Artificial Sequence
  Primer
  misc_feature (16)..(17): n is a, c, g, or t
  misc_feature (19)..(20): n is a, c, g, or t
  misc_feature (22)..(23): n is a, c, g, or t
gctgttgcatctggtnncnncnnagtagcggcagctgggaatga

SEQ ID NO: 450 - DNA, 46 bp, Artificial Sequence
  Primer
  misc_feature (17)..(18): n is a, c, g, or t
  misc_feature (20)..(21): n is a, c, g, or t
  misc_feature (23)..(24): n is a, c, g, or t
cccagctgccgctactnngnngnnaccagatgcaacagctttatca

SEQ ID NO: 451 - DNA, 46 bp, Artificial Sequence
  Primer
  misc_feature (16)..(17): n is a, c, g, or t
  misc_feature (19)..(20): n is a, c, g, or t
  misc_feature (22)..(23): n is a, c, g, or t
gttgcatctggtgtcnncnnannagcggcagctgggaatgagggaa

SEQ ID NO: 452 - DNA, 45 bp, Artificial Sequence
  Primer
  misc_feature (17)..(18): n is a, c, g, or t
  misc_feature (20)..(21): n is a, c, g, or t
  misc_feature (23)..(24): n is a, c, g, or t
attcccagctgccgctnntnngnngacaccagatgcaacagcttt

SEQ ID NO: 453 - DNA, 44 bp, Artificial Sequence
  Primer
  misc_feature (16)..(17): n is a, c, g, or t
  misc_feature (19)..(20): n is a, c, g, or t
  misc_feature (22)..(23): n is a, c, g, or t
gcatctggtgtcgtcnnannannggcagctgggaatgagggaac

SEQ ID NO: 454 - DNA, 44 bp, Artificial Sequence
  Primer
  misc_feature (17)..(18): n is a, c, g, or t
  misc_feature (20)..(21): n is a, c, g, or t
  misc_feature (23)..(24): n is a, c, g, or t
ctcattcccagctgccnntnntnngacgacaccagatgcaacag

SEQ ID NO: 455 - DNA, 44 bp, Artificial Sequence
  Primer
  misc_feature (16)..(17): n is a, c, g, or t
  misc_feature (19)..(20): n is a, c, g, or t
  misc_feature (22)..(23): n is a, c, g, or t
tctggtgtcgtcgtannanngnnagctgggaatgagggaacatc

SEQ ID NO: 456 - DNA, 45 bp, Artificial Sequence
  Primer
  misc_feature (17)..(18): n is a, c, g, or t
  misc_feature (20)..(21): n is a, c, g, or t
  misc_feature (23)..(24): n is a, c, g, or t
tccctcattcccagctnncnntnntacgacgacaccagatgcaac

SEQ ID NO: 457 - DNA, 46 bp, Artificial Sequence
  Primer
  misc_feature (16)..(17): n is a, c, g, or t
  misc_feature (19)..(20): n is a, c, g, or t
  misc_feature (22)..(23): n is a, c, g, or t
ggtgtcgtcgtagtanngnnanntgggaatgagggaacatccggat

SEQ ID NO: 458 - DNA, 46 bp, Artificial Sequence
  Primer
  misc_feature (17)..(18): n is a, c, g, or t
  misc_feature (20)..(21): n is a, c, g, or t
  misc_feature (23)..(24): n is a, c, g, or t
tgttccctcattcccanntnncnntactacgacgacaccagatgca

SEQ ID NO: 459 - DNA, 45 bp, Artificial Sequence
  Primer
  misc_feature (16)..(17): n is a, c, g, or t
  misc_feature (19)..(20): n is a, c, g, or t
  misc_feature (22)..(23): n is a, c, g, or t
gctgggaatgagggannanncnnatcatcgagtaccgtcggttat

SEQ ID NO: 460 - DNA, 47 bp, Artificial Sequence
  Primer
  misc_feature (17)..(18): n is a, c, g, or t
  misc_feature (20)..(21): n is a, c, g, or t
  misc_feature (23)..(24): n is a, c, g, or t
gacggtactcgatgatnngnntnntccctcattcccagctgccgcta

SEQ ID NO: 461 - DNA, 45 bp, Artificial Sequence
  Primer
  misc_feature (16)..(17): n is a, c, g, or t
  misc_feature (19)..(20): n is a, c, g, or t
  misc_feature (22)..(23): n is a, c, g, or t
gggaatgagggaacanncnnannatcgagtaccgtcggttatcca

SEQ ID NO: 462 - DNA, 44 bp, Artificial Sequence
  Primer
  misc_feature (17)..(18): n is a, c, g, or t
  misc_feature (20)..(21): n is a, c, g, or t
  misc_feature (23)..(24): n is a, c, g, or t
accgacggtactcgatnntnngnntgttccctcattcccagctg

SEQ ID NO: 463 - DNA, 44 bp, Artificial Sequence
  Primer
  misc_feature (16)..(17): n is a, c, g, or t
  misc_feature (19)..(20): n is a, c, g, or t
  misc_feature (22)..(23): n is a, c, g, or t
aatgagggaacatccnnannanngagtaccgtcggttatccagg

SEQ ID NO: 464 - DNA, 44 bp, Artificial Sequence
  Primer
  misc_feature (17)..(18): n is a, c, g, or t
  misc_feature (20)..(21): n is a, c, g, or t
  misc_feature (23)..(24): n is a, c, g, or t
ataaccgacggtactcnntnntnnggatgttccctcattcccag

SEQ ID NO: 465 - DNA, 46 bp, Artificial Sequence
  Primer
  misc_feature (16)..(17): n is a, c, g, or t
  misc_feature (19)..(20): n is a, c, g, or t
  misc_feature (22)..(23): n is a, c, g, or t
acatccggatcatcgnntnncnncggttatccaggcaagtaccctt

SEQ ID NO: 466 - DNA, 44 bp, Artificial Sequence
  Primer
  misc_feature (17)..(18): n is a, c, g, or t
  misc_feature (20)..(21): n is a, c, g, or t
  misc_feature (23)..(24): n is a, c, g, or t
cttgcctggataaccgnngnnanncgatgatccggatgttccct

SEQ ID NO: 467 - DNA, 45 bp, Artificial Sequence
  Primer
  misc_feature (16)..(17): n is a, c, g, or t
  misc_feature (19)..(20): n is a, c, g, or t
  misc_feature (22)..(23): n is a, c, g, or t
tccggatcatcgagtnncnncnnttatccaggcaagtacccttca

SEQ ID NO: 468 - DNA, 45 bp, Artificial Sequence
  Primer
  misc_feature (17)..(18): n is a, c, g, or t
  misc_feature (20)..(21): n is a, c, g, or t
  misc_feature (23)..(24): n is a, c, g, or t
gtacttgcctggataanngnngnnactcgatgatccggatgttcc

SEQ ID NO: 469 - DNA, 45 bp, Artificial Sequence
  Primer
  misc_feature (16)..(17): n is a, c, g, or t
  misc_feature (19)..(20): n is a, c, g, or t
  misc_feature (22)..(23): n is a, c, g, or t
tcgagtaccgtcggtnntnnanncaagtacccttcagtgattgca

SEQ ID NO: 470 - DNA, 44 bp, Artificial Sequence
  Primer
  misc_feature (17)..(18): n is a, c, g, or t
  misc_feature (20)..(21): n is a, c, g, or t
  misc_feature (23)..(24): n is a, c, g, or t
cactgaagggtacttgnntnnannaccgacggtactcgatgatc

SEQ ID NO: 471 - DNA, 45 bp, Artificial Sequence
  Primer
  misc_feature (16)..(17): n is a, c, g, or t
  misc_feature (19)..(20): n is a, c, g, or t
  misc_feature (22)..(23): n is a, c, g, or t
agtaccgtcggttatnnanncnngtacccttcagtgattgcagtg

SEQ ID NO: 472 - DNA, 45 bp, Artificial Sequence
  Primer
  misc_feature (17)..(18): n is a, c, g, or t
  misc_feature (20)..(21): n is a, c, g, or t
  misc_feature (23)..(24): n is a, c, g, or t
aatcactgaagggtacnngnntnnataaccgacggtactcgatga

SEQ ID NO: 473 - DNA, 43 bp, Artificial Sequence
  Primer
  misc_feature (16)..(17): n is a, c, g, or t
  misc_feature (19)..(20): n is a, c, g, or t
  misc_feature (22)..(23): n is a, c, g, or t
accgtcggttatccanncnngnncccttcagtgattgcagtgg

SEQ ID NO: 474 - DNA, 45 bp, Artificial Sequence
  Primer
  misc_feature (17)..(18): n is a, c, g, or t
  misc_feature (20)..(21): n is a, c, g, or t
  misc_feature (23)..(24): n is a, c, g, or t
tgcaatcactgaagggnncnngnntggataaccgacggtactcga

SEQ ID NO: 475 - DNA, 45 bp, Artificial Sequence
  Primer
  misc_feature (16)..(17): n is a, c, g, or t
  misc_feature (19)..(20): n is a, c, g, or t
  misc_feature (22)..(23): n is a, c, g, or t
gtcggttatccaggcnngnncnnttcagtgattgcagtgggcgct

SEQ ID NO: 476 - DNA, 44 bp, Artificial Sequence
  Primer
  misc_feature (17)..(18): n is a, c, g, or t
  misc_feature (20)..(21): n is a, c, g, or t
  misc_feature (23)..(24): n is a, c, g, or t
cactgcaatcactgaanngnncnngcctggataaccgacggtac

SEQ ID NO: 477 - DNA, 45 bp, Artificial Sequence
  Primer
  misc_feature (16)..(17): n is a, c, g, or t
  misc_feature (19)..(20): n is a, c, g, or t
  misc_feature (22)..(23): n is a, c, g, or t
ggttatccaggcaagnncnntnnagtgattgcagtgggcgctgta

SEQ ID NO: 478 - DNA, 46 bp, Artificial Sequence
  Primer
  misc_feature (17)..(18): n is a, c, g, or t
  misc_feature (20)..(21): n is a, c, g, or t
  misc_feature (23)..(24): n is a, c, g, or t
gcccactgcaatcactnnanngnncttgcctggataaccgacggta

SEQ ID NO: 479 - DNA, 44 bp, Artificial Sequence
  Primer
  misc_feature (16)..(17): n is a, c, g, or t
  misc_feature (19)..(20): n is a, c, g, or t
  misc_feature (22)..(23): n is a, c, g, or t
tatccaggcaagtacnntnnanngattgcagtgggcgctgtaga

SEQ ID NO: 480 - DNA, 45 bp, Artificial Sequence
  Primer
  misc_feature (17)..(18): n is a, c, g, or t
  misc_feature (20)..(21): n is a, c, g, or t
  misc_feature (23)..(24): n is a, c, g, or t
agcgcccactgcaatcnntnnanngtacttgcctggataaccgac

SEQ ID NO: 481 - DNA, 44 bp, Artificial Sequence
  Primer
  misc_feature (16)..(17): n is a, c, g, or t
  misc_feature (19)..(20): n is a, c, g, or t
  misc_feature (22)..(23): n is a, c, g, or t
gtgggcgctgtagacnntnnanntcaacgtgcctctttttcctc

SEQ ID NO: 482 - DNA, 44 bp, Artificial Sequence
  Primer
  misc_feature (17)..(18): n is a, c, g, or t
  misc_feature (20)..(21): n is a, c, g, or t
  misc_feature (23)..(24): n is a, c, g, or t
aaaagaggcacgttganntnnanngtctacagcgcccactgcaa

SEQ ID NO: 483 - DNA, 44 bp, Artificial Sequence
  Primer
  misc_feature (16)..(17): n is a, c, g, or t
  misc_feature (19)..(20): n is a, c, g, or t
  misc_feature (22)..(23): n is a, c, g, or t
ggcgctgtagactctnnanntnnacgtgcctctttttcctccgt

SEQ ID NO: 484 - DNA, 44 bp, Artificial Sequence
  Primer
  misc_feature (17)..(18): n is a, c, g, or t
  misc_feature (20)..(21): n is a, c, g, or t
  misc_feature (23)..(24): n is a, c, g, or t
ggaaaaagaggcacgtnnanntnnagagtctacagcgcccactg

SEQ ID NO: 485 - DNA, 45 bp, Artificial Sequence
  Primer
  misc_feature (16)..(17): n is a, c, g, or t
  misc_feature (19)..(20): n is a, c, g, or t
  misc_feature (22)..(23): n is a, c, g, or t
gctgtagactcttcanntnnanntgcctctttttcctccgtggga

SEQ ID NO: 486 - DNA, 44 bp, Artificial Sequence
  Primer
  misc_feature (17)..(18): n is a, c, g, or t
  misc_feature (20)..(21): n is a, c, g, or t
  misc_feature (23)..(24): n is a, c, g, or t
ggaggaaaaagaggcanntnnanntgaagagtctacagcgccca

SEQ ID NO: 487 - DNA, 43 bp, Artificial Sequence
  Primer
  misc_feature (16)..(17): n is a, c, g, or t
  misc_feature (19)..(20): n is a, c, g, or t
  misc_feature (22)..(23): n is a, c, g, or t
gtagactcttcaaatnnanntnnctctttttcctccgtgggac

SEQ ID NO: 488 - DNA, 47 bp, Artificial Sequence
  Primer
  misc_feature (17)..(18): n is a, c, g, or t
  misc_feature (20)..(21): n is a, c, g, or t
  misc_feature (23)..(24): n is a, c, g, or t
cacggaggaaaaagagnnanntnnatttgaagagtctacagcgccca

SEQ ID NO: 489 - DNA, 44 bp, Artificial Sequence
  Primer
  misc_feature (16)..(17): n is a, c, g, or t
  misc_feature (19)..(20): n is a, c, g, or t
  misc_feature (22)..(23): n is a, c, g, or t
gactcttcaaatcaanntnncnntttttcctccgtgggaccgga

SEQ ID NO: 490 - DNA, 50 bp, Artificial Sequence
  Primer
  misc_feature (17)..(18): n is a, c, g, or t
  misc_feature (20)..(21): n is a, c, g, or t
  misc_feature (23)..(24): n is a, c, g, or t
tcccacggaggaaaaanngnnannttgatttgaagagtctacagcgccca

SEQ ID NO: 491 - DNA, 45 bp, Artificial Sequence
  Primer
  misc_feature (16)..(17): n is a, c, g, or t
  misc_feature (19)..(20): n is a, c, g, or t
  misc_feature (22)..(23): n is a, c, g, or t
gcctctttttcctccnngnnannggagctggatgtcatggcccct

SEQ ID NO: 492 - DNA, 45 bp, Artificial Sequence
  Primer
  misc_feature (17)..(18): n is a, c, g, or t
  misc_feature (20)..(21): n is a, c, g, or t
  misc_feature (23)..(24): n is a, c, g, or t
catgacatccagctccnntnncnnggaggaaaaagaggcacgttg

SEQ ID NO: 493 - DNA, 45 bp, Artificial Sequence
  Primer
  misc_feature (16)..(17): n is a, c, g, or t
  misc_feature (19)..(20): n is a, c, g, or t
  misc_feature (22)..(23): n is a, c, g, or t
ttttcctccgtggganngnngnnggatgtcatggcccctggcgtt

SEQ ID NO: 494 - DNA, 44 bp, Artificial Sequence
  Primer
  misc_feature (17)..(18): n is a, c, g, or t
  misc_feature (20)..(21): n is a, c, g, or t
  misc_feature (23)..(24): n is a, c, g, or t
aggggccatgacatccnncnncnntcccacggaggaaaaagagg

SEQ ID NO: 495 - DNA, 48 bp, Artificial Sequence
  Primer
  misc_feature (16)..(17): n is a, c, g, or t
  misc_feature (19)..(20): n is a, c, g, or t
  misc_feature (22)..(23): n is a, c, g, or t
tcctccgtgggaccgnngnngnntgtcatggcccctggcgtttctatt

SEQ ID NO: 496 - DNA, 44 bp, Artificial Sequence
  Primer
  misc_feature (17)..(18): n is a, c, g, or t
  misc_feature (20)..(21): n is a, c, g, or t
  misc_feature (23)..(24): n is a, c, g, or t
gccaggggccatgacanncnncnncggtcccacggaggaaaaag

SEQ ID NO: 497 - DNA, 45 bp, Artificial Sequence
  Primer
  misc_feature (16)..(17): n is a, c, g, or t
  misc_feature (19)..(20): n is a, c, g, or t
  misc_feature (22)..(23): n is a, c, g, or t
tccgtgggaccggagnngnntnncatggcccctggcgtttctatt

SEQ ID NO: 498 - DNA, 46 bp, Artificial Sequence
  Primer
  misc_feature (17)..(18): n is a, c, g, or t
  misc_feature (20)..(21): n is a, c, g, or t
  misc_feature (23)..(24): n is a, c, g, or t
aacgccaggggccatgnnanncnnctccggtcccacggaggaaaaa

SEQ ID NO: 499 - DNA, 45 bp, Artificial Sequence
  Primer
  misc_feature (16)..(17): n is a, c, g, or t
  misc_feature (19)..(20): n is a, c, g, or t
  misc_feature (22)..(23): n is a, c, g, or t
gtgggaccggagctgnntnncnnggcccctggcgtttctattcaa

SEQ ID NO: 500 - DNA, 47 bp, Artificial Sequence
  Primer
  misc_feature (17)..(18): n is a, c, g, or t
  misc_feature (20)..(21): n is a, c, g, or t
  misc_feature (23)..(24): n is a, c, g, or t
agaaacgccaggggccnngnnanncagctccggtcccacggaggaaa

SEQ ID NO: 501 - DNA, 46 bp, Artificial Sequence
  Primer
  misc_feature (16)..(17): n is a, c, g, or t
  misc_feature (19)..(20): n is a, c, g, or t
  misc_feature (22)..(23): n is a, c, g, or t
ggaccggagctggatnncnngnnccctggcgtttctattcaatcga

SEQ ID NO: 502 - DNA, 45 bp, Artificial Sequence
  Primer
  misc_feature (17)..(18): n is a, c, g, or t
  misc_feature (20)..(21): n is a, c, g, or t
  misc_feature (23)..(24): n is a, c, g, or t
aatagaaacgccagggnncnngnnatccagctccggtcccacgga

SEQ ID NO: 503 - DNA, 44 bp, Artificial Sequence
  Primer
  misc_feature (16)..(17): n is a, c, g, or t
  misc_feature (19)..(20): n is a, c, g, or t
  misc_feature (22)..(23): n is a, c, g, or t
gtcatggcccctggcnntnntnntcaatcgacgcttccagggaa

SEQ ID NO: 504 - DNA, 44 bp, Artificial Sequence
  Primer
  misc_feature (17)..(18): n is a, c, g, or t
  misc_feature (20)..(21): n is a, c, g, or t
  misc_feature (23)..(24): n is a, c, g, or t
tggaagcgtcgattgannannanngccaggggccatgacatcca

SEQ ID NO: 505 - DNA, 46 bp, Artificial Sequence
  Primer
  misc_feature (16)..(17): n is a, c, g, or t
  misc_feature (19)..(20): n is a, c, g, or t
  misc_feature (22)..(23): n is a, c, g, or t
attcaatcgacgcttnnanngnncaagtatggtgcgcaaaacggga

SEQ ID NO: 506 - DNA, 46 bp, Artificial Sequence
  Primer
  misc_feature (17)..(18): n is a, c, g, or t
  misc_feature (20)..(21): n is a, c, g, or t
  misc_feature (23)..(24): n is a, c, g, or t
ttgcgcaccatacttgnncnntnnaagcgtcgattgaatagaaacg

SEQ ID NO: 507 - DNA, 45 bp, Artificial Sequence
  Primer
  misc_feature (16)..(17): n is a, c, g, or t
  misc_feature (19)..(20): n is a, c, g, or t
  misc_feature (22)..(23): n is a, c, g, or t
caatcgacgcttccanngnncnngtatggtgcgcaaaacgggact

SEQ ID NO: 508 - DNA, 46 bp, Artificial Sequence
  Primer
  misc_feature (17)..(18): n is a, c, g, or t
  misc_feature (20)..(21): n is a, c, g, or t
  misc_feature (23)..(24): n is a, c, g, or t
gttttgcgcaccatacnngnncnntggaagcgtcgattgaatagaa

SEQ ID NO: 509 - DNA, 48 bp, Artificial Sequence
  Primer
  misc_feature (16)..(17): n is a, c, g, or t
  misc_feature (19)..(20): n is a, c, g, or t
  misc_feature (22)..(23): n is a, c, g, or t
gggaacaagtatggtnngnnanncgggacttccatggcctcgccgcat

SEQ ID NO: 510 - DNA, 45 bp, Artificial Sequence
  Primer
  misc_feature (17)..(18): n is a, c, g, or t
  misc_feature (20)..(21): n is a, c, g, or t
  misc_feature (23)..(24): n is a, c, g, or t
ggccatggaagtcccgnntnncnnaccatacttgttccctggaag

SEQ ID NO: 511 - DNA, 45 bp, Artificial Sequence
  Primer
  misc_feature (16)..(17): n is a, c, g, or t
  misc_feature (19)..(20): n is a, c, g, or t
  misc_feature (22)..(23): n is a, c, g, or t
aacaagtatggtgcgnnanncnngacttccatggcctcgccgcat

SEQ ID NO: 512 - DNA, 44 bp, Artificial Sequence
  Primer
  misc_feature (17)..(18): n is a, c, g, or t
  misc_feature (20)..(21): n is a, c, g, or t
  misc_feature (23)..(24): n is a, c, g, or t
cgaggccatggaagtcnngnntnncgcaccatacttgttccctg

SEQ ID NO: 513 - DNA, 43 bp, Artificial Sequence
  Primer
  misc_feature (16)..(17): n is a, c, g, or t
  misc_feature (19)..(20): n is a, c, g, or t
  misc_feature (22)..(23): n is a, c, g, or t
aagtatggtgcgcaanncnngnnttccatggcctcgccgcatg

SEQ ID NO: 514 - DNA, 45 bp, Artificial Sequence
  Primer
  misc_feature (17)..(18): n is a, c, g, or t
  misc_feature (20)..(21): n is a, c, g, or t
  misc_feature (23)..(24): n is a, c, g, or t
cggcgaggccatggaanncnngnnttgcgcaccatacttgttccc

SEQ ID NO: 515 - DNA, 43 bp, Artificial Sequence
  Primer
  misc_feature (16)..(17): n is a, c, g, or t
  misc_feature (19)..(20): n is a, c, g, or t
  misc_feature (22)..(23): n is a, c, g, or t
tatggtgcgcaaaacnngnntnncatggcctcgccgcatgtag

SEQ ID NO: 516 - DNA, 46 bp, Artificial Sequence
  Primer
  misc_feature (17)..(18): n is a, c, g, or t
  misc_feature (20)..(21): n is a, c, g, or t
  misc_feature (23)..(24): n is a, c, g, or t
atgcggcgaggccatgnnanncnngttttgcgcaccatacttgttc

SEQ ID NO: 517 - DNA, 47 bp, Artificial Sequence
  Primer
  misc_feature (16)..(17): n is a, c, g, or t
  misc_feature (19)..(20): n is a, c, g, or t
  misc_feature (22)..(23): n is a, c, g, or t
ccgcatgtagctgggnngnncnnattgattctttctaagcacccgaa

SEQ ID NO: 518 - DNA, 48 bp, Artificial Sequence
  Primer
  misc_feature (17)..(18): n is a, c, g, or t
  misc_feature (20)..(21): n is a, c, g, or t
  misc_feature (23)..(24): n is a, c, g, or t
cttagaaagaatcaatnngnncnncccagctacatgcggcgaggccat

SEQ ID NO: 519 - DNA, 46 bp, Artificial Sequence
  Primer
  misc_feature (16)..(17): n is a, c, g, or t
  misc_feature (19)..(20): n is a, c, g, or t
  misc_feature (22)..(23): n is a, c, g, or t
catgtagctggggcgnncnnanngattctttctaagcacccgaact

SEQ ID NO: 520 - DNA, 51 bp, Artificial Sequence
  Primer
  misc_feature (17)..(18): n is a, c, g, or t
  misc_feature (20)..(21): n is a, c, g, or t
  misc_feature (23)..(24): n is a, c, g, or t
gtgcttagaaagaatcnntnngnncgccccagctacatgcggcgaggccat

SEQ ID NO: 521 - DNA, 44 bp, Artificial Sequence
  Primer
  misc_feature (16)..(17): n is a, c, g, or t
  misc_feature (19)..(20): n is a, c, g, or t
  misc_feature (22)..(23): n is a, c, g, or t
gtagctggggcggccnnanngnntctttctaagcacccgaactg

SEQ ID NO: 522 - DNA, 43 bp, Artificial Sequence
  Primer
  misc_feature (17)..(18): n is a, c, g, or t
  misc_feature (20)..(21): n is a, c, g, or t
  misc_feature (23)..(24): n is a, c, g, or t
cgggtgcttagaaaganncnntnnggccgccccagctacatgc

SEQ ID NO: 523 - DNA, 46 bp, Artificial Sequence
  Primer
  misc_feature (16)..(17): n is a, c, g, or t
  misc_feature (19)..(20): n is a, c, g, or t
  misc_feature (22)..(23): n is a, c, g, or t
ttgattctttctaagnncnngnnctggacaaacactcaagtccgca

SEQ ID NO: 524 - DNA, 45 bp, Artificial Sequence
  Primer
  misc_feature (17)..(18): n is a, c, g, or t
  misc_feature (20)..(21): n is a, c, g, or t
  misc_feature (23)..(24): n is a, c, g, or t
ttgagtgtttgtccagnncnngnncttagaaagaatcaatgcggc

SEQ ID NO: 525 - DNA, 45 bp, Artificial Sequence
  Primer
  misc_feature (16)..(17): n is a, c, g, or t
  misc_feature (19)..(20): n is a, c, g, or t
  misc_feature (22)..(23): n is a, c, g, or t
ctttctaagcacccgnncnngnnaaacactcaagtccgcagcagt

SEQ ID NO: 526 - DNA, 46 bp, Artificial Sequence
  Primer
  misc_feature (17)..(18): n is a, c, g, or t
  misc_feature (20)..(21): n is a, c, g, or t
  misc_feature (23)..(24): n is a, c, g, or t
gcggacttgagtgtttnncnngnncgggtgcttagaaagaatcaat

SEQ ID NO: 527 - DNA, 48 bp, Artificial Sequence
  Primer
  misc_feature (16)..(17): n is a, c, g, or t
  misc_feature (19)..(20): n is a, c, g, or t
  misc_feature (22)..(23): n is a, c, g, or t
tggacaaacactcaanncnncnncagtttagaaaacaccactacaaaa

SEQ ID NO: 528 - DNA, 47 bp, Artificial Sequence
  Primer
  misc_feature (17)..(18): n is a, c, g, or t
  misc_feature (20)..(21): n is a, c, g, or t
  misc_feature (23)..(24): n is a, c, g, or t
ggtgttttctaaactgnngnngnnttgagtgtttgtccagttcgggt

SEQ ID NO: 529 - DNA, 47 bp, Artificial Sequence
  Primer
  misc_feature (16)..(17): n is a, c, g, or t
  misc_feature (19)..(20): n is a, c, g, or t
  misc_feature (22)..(23): n is a, c, g, or t
ttagaaaacaccactnnannanntggtgattctttctactatggaaa

SEQ ID NO: 530 - DNA, 46 bp, Artificial Sequence
  Primer
  misc_feature (17)..(18): n is a, c, g, or t
  misc_feature (20)..(21): n is a, c, g, or t
  misc_feature (23)..(24): n is a, c, g, or t
gtagaaagaatcaccanntnntnnagtggtgttttctaaactgctg

SEQ ID NO: 531 - DNA, 46 bp, Artificial Sequence
  Primer
  misc_feature (16)..(17): n is a, c, g, or t
  misc_feature (19)..(20): n is a, c, g, or t
  misc_feature (22)..(23): n is a, c, g, or t
accactacaaaacttnntnntnntttctactatggaaaagggctga

SEQ ID NO: 532 - DNA, 48 bp, Artificial Sequence
  Primer
  misc_feature (17)..(18): n is a, c, g, or t
  misc_feature (20)..(21): n is a, c, g, or t
  misc_feature (23)..(24): n is a, c, g, or t
ttttccatagtagaaannannannaagttttgtagtggtgttttctaa

SEQ ID NO: 533 - DNA, 45 bp, Artificial Sequence
  Primer
  misc_feature (16)..(17): n is a, c, g, or t
  misc_feature (19)..(20): n is a, c, g, or t
  misc_feature (22)..(23): n is a, c, g, or t
gattctttctactatnnannanngctgatcaacgtacaggcggca

SEQ ID NO: 534 - DNA, 48 bp, Artificial Sequence
  Primer
  misc_feature (17)..(18): n is a, c, g, or t
  misc_feature (20)..(21): n is a, c, g, or t
  misc_feature (23)..(24): n is a, c, g, or t
ctgtacgttgatcagcnntnntnnatagtagaaagaatcaccaagttt

SEQ ID NO: 535 - DNA, 42 bp, Artificial Sequence
  Primer
tcaaggctacaatggagcaaatgttaaagtagcggttatcga

SEQ ID NO: 536 - DNA, 38 bp, Artificial Sequence
  Primer
tttaacatttgctccattgtagccttgagagtgcagag

SEQ ID NO: 537 - DNA, 38 bp, Artificial Sequence
  Primer
ctacactggaggaggtgttaaagtagcggttatcgaca

SEQ ID NO: 538 - DNA, 37 bp, Artificial Sequence
  Primer
ctactttaacacctcctccagtgtagccttgagagtg

SEQ ID NO: 539 - DNA, 40 bp, Artificial Sequence
  Primer
aggctacactggaagaaatgttaaagtagcggttatcgac

SEQ ID NO: 540 - DNA, 34 bp, Artificial Sequence
  Primer
ctttaacatttcttccagtgtagccttgagagtg

SEQ ID NO: 541 - DNA, 42 bp, Artificial Sequence
  Primer
aaggctacactgcaggaggtgttaaagtagcggttatcgaca

SEQ ID NO: 542 - DNA, 40 bp, Artificial Sequence
  Primer
ctactttaacacctcctgcagtgtagccttgagagtgcag

SEQ ID NO: 543 - DNA, 37 bp, Artificial Sequence
  Primer
cgtttcaagatccctcttctcatggcacacacgtcgc

SEQ ID NO: 544 - DNA, 40 bp, Artificial Sequence
  Primer
tgtgccatgagaagagggatcttgaaacgggtttgtttcg

SEQ ID NO: 545 - DNA, 38 bp, Artificial Sequence
  Primer
tgccgtccgaaccaaacccgtttcaagataacaattct

SEQ ID NO: 546 - DNA, 37 bp, Artificial Sequence
  Primer
tcttgaaacgggtttggttcggacggcaccatagaag

SEQ ID NO: 547 - DNA, 40 bp, Artificial Sequence
  Primer
ccgtttcaagatcccaatcatcatggcacacacgtcgcag

SEQ ID NO: 548 - DNA, 42 bp, Artificial Sequence
  Primer
tgtgtgccatgatgattgggatcttgaaacgggtttgtttcg

SEQ ID NO: 549 - DNA, 45 bp, Artificial Sequence
  Primer
acaaacccgttttcagatcccaattctcatggcacacacgtcgca

SEQ ID NO: 550 - DNA, 43 bp, Artificial Sequence
  Primer
ccatgagaattgggatctgaaaacgggtttgtttcggacggca

SEQ ID NO: 551 - DNA, 38 bp, Artificial Sequence
  Primer
ggttgcggcgtcatacaattctattggcgtgcttggtg

SEQ ID NO: 552 - DNA, 38 bp, Artificial Sequence
  Primer
gccaatagaattgtatgacgccgcaaccgttcctgcga

SEQ ID NO: 553 - DNA, 40 bp, Artificial Sequence
  Primer
tggtgtagcctcgggtgtttcgctctacgccgttaaagtt

SEQ ID NO: 554 - DNA, 39 bp, Artificial Sequence
  Primer
cgtagagcgaaacacccgaggctacaccaagcacgccaa

SEQ ID NO: 555 - DNA, 42 bp, Artificial Sequence
  Primer
gtgtagccccgggtgttgcactctacgccgttaaagttcttg

SEQ ID NO: 556 - DNA, 43 bp, Artificial Sequence
  Primer
acggcgtagagtgcaacacccggggctacaccaagcacgccaa

SEQ ID NO: 557 - DNA, 44 bp, Artificial Sequence
  Primer
tggtgtagccccgactcttggactctacgccgttaaagttcttg

SEQ ID NO: 558 - DNA, 43 bp, Artificial Sequence
  Primer
acggcgtagagtccaagagtcggggctacaccaagcacgccaa

SEQ ID NO: 559 - DNA, 41 bp, Artificial Sequence
  Primer
gcctgggagcacaaggctctagtgcggcacttaaagcagca

SEQ ID NO: 560 - DNA, 41 bp, Artificial Sequence
  Primer
agtgccgcactagagccttgtgctcccaggctcatgttgat

SEQ ID NO: 561 - DNA, 37 bp, Artificial Sequence
  Primer
atggcccctggctattctattcaatcgacgcttccag

SEQ ID NO: 562 - DNA, 36 bp, Artificial Sequence
  Primer
tcgattgaatagaatagccaggggccatgacatcca

SEQ ID NO: 563 - DNA, 42 bp, Artificial Sequence
  Primer
tcgacgcttccaaggtccgtgtatggtgcgcaaaacgggact

SEQ ID NO: 564 - DNA, 44 bp, Artificial Sequence
  Primer
ttgcgcaccatacacggaccttggaagcgtcgattgaatagaaa

SEQ ID NO: 565 - DNA, 39 bp, Artificial Sequence
  Primer
catggcacacactgcggaggaacggttgcggcgttaaac

SEQ ID NO: 566 - DNA, 39 bp, Artificial Sequence
  Primer
gcaaccgttcctccgcagtgtgtgccatgagaattgtta

SEQ ID NO: 567 - DNA, 43 bp, Artificial Sequence
  Primer
gtcgcaggaacgattggttcaaacaattctattggcgtgcttg

SEQ ID NO: 568 - DNA, 45 bp, Artificial Sequence
  Primer
caatagaattgtttgaaccaatcgttcctgcgacgtgtgtgccat

SEQ ID NO: 569 - DNA, 41 bp, Artificial Sequence
  Primer
aacggttgcggcgcatggaaattctattggcgtgcttggtg

SEQ ID NO: 570 - DNA, 41 bp, Artificial Sequence
  Primer
caatagaatttccatgcgccgcaaccgttcctgcgacgtgt

SEQ ID NO: 571 - DNA, 43 bp, Artificial Sequence
  Primer
aacggttgcggcgagaggaggttctattggcgtgcttggtgta

SEQ ID NO: 572 - DNA, 46 bp, Artificial Sequence
  Primer
cacgccaatagaacctcctctcgccgcaaccgttcctgcgacgtgt

SEQ ID NO: 573 - DNA, 43 bp, Artificial Sequence
  Primer
aacggttgcggcgggaggcggttctattggcgtgcttggtgta

SEQ ID NO: 574 - DNA, 46 bp, Artificial Sequence
  Primer
cacgccaatagaaccgcctcccgccgcaaccgttcctgcgacgtgt

SEQ ID NO: 575 - DNA, 37 bp, Artificial Sequence
  Primer
tgcttcgctctacggcgttaaagttcttgcagcagac

SEQ ID NO: 576 - DNA, 39 bp, Artificial Sequence
  Primer
caagaactttaacgccgtagagcgaagcagacggggcta

SEQ ID NO: 577 - DNA, 43 bp, Artificial Sequence
  Primer
ttcgctctacgcctcatgttctgcagcagacggatcaggccaa

SEQ ID NO: 578 - DNA, 42 bp, Artificial Sequence
  Primer
atccgtctgctgcagaacatgaggcgtagagcgaagcagacg

SEQ ID NO: 579 - DNA, 41 bp, Artificial Sequence
  Primer
aataacatggatatatcttgcatgagcctgggagcaccaag

SEQ ID NO: 580 - DNA, 44 bp, Artificial Sequence
  Primer
caggctcatgcaagatatatccatgttattcgcgatggcccatt

SEQ ID NO: 581 - DNA, 43 bp, Artificial Sequence
  Primer
cgaataacatggatcttatctgcatgagcctgggagcaccaag

SEQ ID NO: 582 - DNA, 45 bp, Artificial Sequence
  Primer
ccaggctcatgcagataagatccatgttattcgcgatggcccatt

SEQ ID NO: 583 - DNA, 44 bp, Artificial Sequence
  Primer
taacatggatgtatgctcattgagcctgggagcaccaagcggca

SEQ ID NO: 584 - DNA, 43 bp, Artificial Sequence
  Primer
tgctcccaggctcaatgagcatacatccatgttattcgcgatg

SEQ ID NO: 585 - DNA, 37 bp, Artificial Sequence
  Primer
acatggatgtaatctgcatgagcctgggagcaccaag

SEQ ID NO: 586 - DNA, 39 bp, Artificial Sequence
  Primer
tcccaggctcatgcagattacatccatgttattcgcgat

SEQ ID NO: 587 - DNA, 38 bp, Artificial Sequence
  Primer
ggatgtaatcaacatcagcctgggagcaccaagcggca

SEQ ID NO: 588 - DNA, 38 bp, Artificial Sequence
  Primer
tgctcccaggctgatgttgattacatccatgttattcg

SEQ ID NO: 589 - DNA, 38 bp, Artificial Sequence
  Primer
ggatgtaatcaacgtaagcctgggagcaccaagcggca

SEQ ID NO: 590 - DNA, 38 bp, Artificial Sequence
  Primer
tgctcccaggcttacgttgattacatccatgttattcg

SEQ ID NO: 591 - DNA, 41 bp, Artificial Sequence
  Primer
ggatgtaatcaacgtaagcgcgggagcaccaagcggcagtg

SEQ ID NO: 592 - DNA, 42 bp, Artificial Sequence
  Primer
ttggtgctcccgcgcttacgttgattacatccatgttattcg

SEQ ID NO: 593 - DNA, 42 bp, Artificial Sequence
  Primer
aatcaacatgagcttcggagcaagcggcagtgcggcacttaa

SEQ ID NO: 594 - DNA, 42 bp, Artificial Sequence
  Primer
cactgccgcttgctccgaagctcatgttgattacatccatgt

SEQ ID NO: 595 - DNA, 40 bp, Artificial Sequence
  Primer
aacatgagcctgtacgcaccaagcggcagtgcggcactta

SEQ ID NO: 596 - DNA, 41 bp, Artificial Sequence
  Primer
cactgccgcttggtgcgtacaggctcatgttgattacatcc

SEQ ID NO: 597 - DNA, 43 bp, Artificial Sequence
  Primer
caacatgagcctgtcagcagatagcggcagtgcggcacttaaa

SEQ ID NO: 598 - DNA, 42 bp, Artificial Sequence
  Primer
gcactgccgctatctgctgacaggctcatgttgattacatcc

SEQ ID NO: 599 - DNA, 43 bp, Artificial Sequence
  Primer
caacatgagcctgaacgcacgtagcggcagtgcggcacttaaa

SEQ ID NO: 600 - DNA, 42 bp, Artificial Sequence
  Primer
gcactgccgctacgtgcgttcaggctcatgttgattacatcc

SEQ ID NO: 601 - DNA, 42 bp, Artificial Sequence
  Primer
atgagcctgggaaattcatctagcggcagtgcggcacttaaa

SEQ ID NO: 602 - DNA, 41 bp, Artificial Sequence
  Primer
gcactgccgctagatgaatttcccaggctcatgttgattac

SEQ ID NO: 603 - DNA, 40 bp, Artificial Sequence
  Primer
catgagcctgggatcagttagcggcagtgcggcacttaaa

SEQ ID NO: 604 - DNA, 38 bp, Artificial Sequence
  Primer
gcactgccgctaactgatcccaggctcatgttgattac

SEQ ID NO: 605 - DNA, 40 bp, Artificial Sequence
  Primer
catgagcctgggatcagatagcggcagtgcggcacttaaa

SEQ ID NO: 606 - DNA, 38 bp, Artificial Sequence
  Primer
gcactgccgctatctgatcccaggctcatgttgattac

SEQ ID NO: 607 - DNA, 40 bp, Artificial Sequence
  Primer
catgagcctgggatcaggtagcggcagtgcggcacttaaa

SEQ ID NO: 608 - DNA, 38 bp, Artificial Sequence
  Primer
gcactgccgctacctgatcccaggctcatgttgattac

SEQ ID NO: 609 - DNA, 40 bp, Artificial Sequence
  Primer
catgagcctgggacactatagcggcagtgcggcacttaaa

SEQ ID NO: 610 - DNA, 38 bp, Artificial Sequence
  Primer
gcactgccgctatagtgtcccaggctcatgttgattac

SEQ ID NO: 611 - DNA, 36 bp, Artificial Sequence
  Primer
gagcctgggagcagacagcggcagtgcggcacttaa

SEQ ID NO: 612 - DNA, 39 bp, Artificial Sequence
  Primer
tgccgcactgccgctgtctgctcccaggctcatgttgat

SEQ ID NO: 613 - DNA, 36 bp, Artificial Sequence
  Primer
gagcctgggagcagaaagcggcagtgcggcacttaa

SEQ ID NO: 614 - DNA, 39 bp, Artificial Sequence
  Primer
tgccgcactgccgctttctgctcccaggctcatgttgat

SEQ ID NO: 615 - DNA, 36 bp, Artificial Sequence
  Primer
gagcctgggagcagtaagcggcagtgcggcacttaa

SEQ ID NO: 616 - DNA, 39 bp, Artificial Sequence
  Primer
tgccgcactgccgcttactgctcccaggctcatgttgat

SEQ ID NO: 617 - DNA, 36 bp, Artificial Sequence
  Primer
gagcctgggagcaggaggcagtgcggcacttaaagc

SEQ ID NO: 618 - DNA, 38 bp, Artificial Sequence
  Primer
agtgccgcactgcctcctgctcccaggctcatgttgat

SEQ ID NO: 619 - DNA, 42 bp, Artificial Sequence
  Primer
agcctgggagcacacggcaatgcggcacttaaagcagcagtt

SEQ ID NO: 620 - DNA, 42 bp, Artificial Sequence
  Primer
tttaagtgccgcattgccgtgtgctcccaggctcatgttgat

SEQ ID NO: 621 - DNA, 38 bp, Artificial Sequence
  Primer
aagcggcagtgcgacacttaaagcagcagttgataaag

SEQ ID NO: 622 - DNA, 38 bp, Artificial Sequence
  Primer
aactgctgctttaagtgtcgcactgccgcttggtgctc

SEQ ID NO: 623 - DNA, 41 bp, Artificial Sequence
  Primer
gttaaagttcttcgtggttgtgacggatcaggccaatactc

SEQ ID NO: 624 - DNA, 41 bp, Artificial Sequence
  Primer
ctgatccgtcacaaccacgaagaactttaacggcgtagagc

SEQ ID NO: 625 - DNA, 40 bp, Artificial Sequence
  Primer
ttaaagttcttgcaggaggcggatcaggccaatactcatg

SEQ ID NO: 626 - DNA, 42 bp, Artificial Sequence
  Primer
tattggcctgatccgcctcctgcaagaactttaacggcgtag

SEQ ID NO: 627 - DNA, 41 bp, Artificial Sequence
  Primer
ttaaagttcttgcaggacgtgacggatcaggccaatactca

SEQ ID NO: 628 - DNA, 38 bp, Artificial Sequence
  Primer
ctgatccgtcacgtcctgcaagaactttaacggcgtag

SEQ ID NO: 629 - DNA, 40 bp, Artificial Sequence
  Primer
ttaaagttcttgcagacggcggatcaggccaatactcatg

SEQ ID NO: 630 - DNA, 42 bp, Artificial Sequence
  Primer
tattggcctgatccgccgtctgcaagaactttaacggcgtag

SEQ ID NO: 631 - DNA, 45 bp, Artificial Sequence
  Primer
taaagttcttgcacatggagattcaggccaatactcatggattat

SEQ ID NO: 632 - DNA, 44 bp, Artificial Sequence
  Primer
agtattggcctgaatctccatgtgcaagaactttaacggcgtag

SEQ ID NO: 633 - DNA, 40 bp, Artificial Sequence
  Primer
aagttcttgcagcacgtaacggatcaggccaatactcatg

SEQ ID NO: 634 - DNA, 44 bp, Artificial Sequence
  Primer
tattggcctgatccgttacgtgctgcaagaactttaacggcgta

SEQ ID NO: 635 - DNA, 45 bp, Artificial Sequence
  Primer
agttcttgcagcagtaggagatggccaatactcatggattatcaa

SEQ ID NO: 636 - DNA, 45 bp, Artificial Sequence
  Primer
tgagtattggccatctcctactgctgcaagaactttaacggcgta

SEQ ID NO: 637 - DNA, 43 bp, Artificial Sequence
  Primer
ttaaagttcttgcagcatgtagcggatcaggccaatactcatg

SEQ ID NO: 638 - DNA, 44 bp, Artificial Sequence
  Primer
tattggcctgatccgctacatgctgcaagaactttaacggcgta

SEQ ID NO: 639 - DNA, 43 bp, Artificial Sequence
  Primer
aagttcttgcagcagactcttcaggccaatactcatggattat

SEQ ID NO: 640 - DNA, 41 bp, Artificial Sequence
  Primer
atgagtattggcctgaagagtctgctgcaagaactttaacg

SEQ ID NO: 641 - DNA, 42 bp, Artificial Sequence
  Primer
ttcttgcagcagactctgtaggccaatactcatggattatca

SEQ ID NO: 642 - DNA, 42 bp, Artificial Sequence
  Primer
catgagtattggcctacagagtctgctgcaagaactttaacg

SEQ ID NO: 643 - DNA, 43 bp, Artificial Sequence
  Primer
aagttcttgcagcagacgattcaggccaatactcatggattat

SEQ ID NO: 644 - DNA, 41 bp, Artificial Sequence
  Primer
atgagtattggcctgaatcgtctgctgcaagaactttaacg

SEQ ID NO: 645 - DNA, 43 bp, Artificial Sequence
  Primer
aagttcttgcagcagacaattcaggccaatactcatggattat

SEQ ID NO: 646 - DNA, 41 bp, Artificial Sequence
  Primer
atgagtattggcctgaattgtctgctgcaagaactttaacg

SEQ ID NO: 647 - DNA, 42 bp, Artificial Sequence
  Primer
ttcttgcagcagacaatctaggccaatactcatggattatca

SEQ ID NO: 648 - DNA, 42 bp, Artificial Sequence
  Primer
catgagtattggcctagattgtctgctgcaagaactttaacg

SEQ ID NO: 649 - DNA, 43 bp, Artificial Sequence
  Primer
ttcttgcagcagacggaggaggccaatactcatggattatcaa

SEQ ID NO: 650 - DNA, 38 bp, Artificial Sequence
  Primer
atgagtattggcctcctccgtctgctgcaagaacttta

SEQ ID NO: 651 - DNA, 43 bp, Artificial Sequence
  Primer
ttcttgcagcagacggagatggccaatactcatggattatcaa

SEQ ID NO: 652 - DNA, 38 bp, Artificial Sequence
  Primer
atgagtattggccatctccgtctgctgcaagaacttta

SEQ ID NO: 653 - DNA, 45 bp, Artificial Sequence
  Primer
tgcagcagacggagtaggcaactactcatggattatcaacggcat

SEQ ID NO: 654 - DNA, 45 bp, Artificial Sequence
  Primer
ataatccatgagtagttgcctactccgtctgctgcaagaacttta

SEQ ID NO: 655 - DNA, 43 bp, Artificial Sequence
  Primer
ttcttgcagcagacggacgtggccaatactcatggattatcaa

SEQ ID NO: 656 - DNA, 38 bp, Artificial Sequence
  Primer
atgagtattggccacgtccgtctgctgcaagaacttta

SEQ ID NO: 657 - DNA, 43 bp, Artificial Sequence
  Primer
aatgggccatctctggtagaatggatgtaatcaacatgagcct

SEQ ID NO: 658 - DNA, 42 bp, Artificial Sequence
  Primer
gattacatccattctaccagagatggcccattcgatgccgtt

SEQ ID NO: 659 - DNA, 40 bp, Artificial Sequence
  Primer
aatgggccatcggacgtaacatggatgtaatcaacatgag

SEQ ID NO: 660 - DNA, 42 bp, Artificial Sequence
  Primer
gattacatccatgttacgtccgatggcccattcgatgccgtt

SEQ ID NO: 661 - DNA, 43 bp, Artificial Sequence
  Primer
aatgggccatcaattctggaatggatgtaatcaacatgagcct

SEQ ID NO: 662 - DNA, 42 bp, Artificial Sequence
  Primer
gattacatccattccagaattgatggcccattcgatgccgtt

SEQ ID NO: 663 - DNA, 36 bp, Artificial Sequence
  Primer
aaaacgggacttcccaggcctcgccgcatgtagctg

SEQ ID NO: 664 - DNA, 38 bp, Artificial Sequence
  Primer
tacatgcggcgaggcctgggaagtcccgttttgcgcac

SEQ ID NO: 665 - DNA, 40 bp, Artificial Sequence
  Primer
aaggctacactggaagaaatgttaaagtagcggttatcga

SEQ ID NO: 666 - DNA, 37 bp, Artificial Sequence
  Primer
ctactttaacatttcttccagtgtagccttgagagtg

SEQ ID NO: 667 - DNA, 38 bp, Artificial Sequence
  Primer
ctacactggatcatatgttaaagtagcggttatcgaca

SEQ ID NO: 668 - DNA, 40 bp, Artificial Sequence
  Primer
taaccgctactttaacatatgatccagtgtagccttgaga

SEQ ID NO: 669 - DNA, 36 bp, Artificial Sequence
  Primer
cttctatggtggattccgaaacaaacccgtttcaag

SEQ ID NO: 670 - DNA, 36 bp, Artificial Sequence
  Primer
ggtttgtttcggaatccaccatagaagcccctccag

SEQ ID NO: 671 - DNA, 39 bp, Artificial Sequence
  Primer
tttcaagataacaatacacatggcacacacgtcgcagga

SEQ ID NO: 672 - DNA, 38 bp, Artificial Sequence
  Primer
tgtgtgccatgtgtattgttatcttgaaacgggtttgt

SEQ ID NO: 673 - DNA, 34 bp, Artificial Sequence
  Primer
gtttcaagatgaaaattctcatggcacacacgtc

SEQ ID NO: 674 - DNA, 40 bp, Artificial Sequence
  Primer
tgtgccatgagaattttcatcttgaaacgggtttgtttcg

SEQ ID NO: 675 - DNA, 39 bp, Artificial Sequence
  Primer
aacccgtttcaagatccaaattctcatggcacacacgtc

SEQ ID NO: 676 - DNA, 38 bp, Artificial Sequence
  Primer
tgccatgagaatttggatcttgaaacgggtttgtttcg

SEQ ID NO: 677 - DNA, 41 bp, Artificial Sequence
  Primer
gtttcaagataaccaatctcatggcacacacgtcgcaggaa

SEQ ID NO: 678 - DNA, 40 bp, Artificial Sequence
  Primer
tgtgtgccatgagattggttatcttgaaacgggtttgttt

SEQ ID NO: 679 - DNA, 41 bp, Artificial Sequence
  Primer
gtttcaagataacgattctcatggcacacacgtcgcaggaa

SEQ ID NO: 680 - DNA, 40 bp, Artificial Sequence
  Primer
tgtgtgccatgagaatcgttatcttgaaacgggtttgttt

SEQ ID NO: 681 - DNA, 36 bp, Artificial Sequence
  Primer
tcaagataacaatcaacatggcacacacgtcgcagg

SEQ ID NO: 682 - DNA, 40 bp, Artificial Sequence
  Primer
acgtgtgtgccatgttgattgttatcttgaaacgggtttg

SEQ ID NO: 683 - DNA, 38 bp, Artificial Sequence
  Primer
tcatggcacacacgcagcaggaacggttgcggcgttaa

SEQ ID NO: 684 - DNA, 38 bp, Artificial Sequence
  Primer
caaccgttcctgctgcgtgtgtgccatgagaattgtta

SEQ ID NO: 685 - DNA, 33 bp, Artificial Sequence
  Primer
tgtagccccggatgcttcgctctacgccgttaa

SEQ ID NO: 686 - DNA, 35 bp, Artificial Sequence; identical to SEQ ID NO: 174
  Primer

SEQ ID NO: 687 - DNA, 36 bp, Artificial Sequence
  Primer
cgttaaagttacagcagcagacggatcaggccaata

SEQ ID NO: 688 - DNA, 40 bp, Artificial Sequence
  Primer
tgatccgtctgctgctgtaactttaacggcgtagagcgaa

SEQ ID NO: 689 - DNA, 36 bp, Artificial Sequence
  Primer
taatcaacatgagcgcgggagcaccaagcggcagtg

SEQ ID NO: 690 - DNA, 35 bp, Artificial Sequence
  Primer
ttggtgctcccgcgctcatgttgattacatccatg

SEQ ID NO: 691 - DNA, 36 bp, Artificial Sequence
  Primer
taatcaacatgagcacgggagcaccaagcggcagtg

SEQ ID NO: 692 - DNA, 35 bp, Artificial Sequence
  Primer
ttggtgctcccgtgctcatgttgattacatccatg

SEQ ID NO: 693 - DNA, 38 bp, Artificial Sequence
  Primer
atgtaatcaacatggcactgggagcaccaagcggcagt

SEQ ID NO: 694 - DNA, 40 bp, Artificial Sequence
  Primer
ttggtgctcccagtgccatgttgattacatccatgttatt

SEQ ID NO: 695 - DNA, 34 bp, Artificial Sequence
  Primer
tgggagcaccaccaggcagtgcggcacttaaagc

SEQ ID NO: 696 - DNA, 36 bp, Artificial Sequence
  Primer
gtgccgcactgcctggtggtgctcccaggctcatgt

SEQ ID NO: 697 - DNA, 37 bp, Artificial Sequence
  Primer
tgagcctgggagcacttagcggcagtgcggcacttaa

SEQ ID NO: 698 - DNA, 39 bp, Artificial Sequence
  Primer
tgccgcactgccgctaagtgctcccaggctcatgttgat

SEQ ID NO: 699 - DNA, 37 bp, Artificial Sequence
  Primer
tgagcctgggagcagaaagcggcagtgcggcacttaa

SEQ ID NO: 700 - DNA, 39 bp, Artificial Sequence; identical to SEQ ID NO: 614
  Primer

SEQ ID NO: 701 - DNA, 37 bp, Artificial Sequence
  Primer
tgagcctgggagcatctagcggcagtgcggcacttaa

SEQ ID NO: 702 - DNA, 39 bp, Artificial Sequence
  Primer
tgccgcactgccgctagatgctcccaggctcatgttgat

SEQ ID NO: 703 - DNA, 35 bp, Artificial Sequence
  Primer
gactcgagccatgaagatcttaaagtcgctggagg

SEQ ID NO: 704 - DNA, 36 bp, Artificial Sequence
  Primer
gactttaagatcttcatggctcgagtcgataccgct

SEQ ID NO: 705 - DNA, 40 bp, Artificial Sequence
  Primer
gcagtccgtgcctcaaggcgtatcacaaattaaagcccct

SEQ ID NO: 706 - DNA, 40 bp, Artificial Sequence
  Primer
atttgtgatacgccttgaggcacggactgcgcgtacgcat

SEQ ID NO: 707 - DNA, 40 bp, Artificial Sequence
  Primer
cagacggatcagcacaatactcatggattatcaacggcat

SEQ ID NO: 708 - DNA, 40 bp, Artificial Sequence
  Primer
taatccatgagtattgtgctgatccgtctgctgcaagaac

SEQ ID NO: 709 - DNA, 38 bp, Artificial Sequence
  Primer
gcagcagacggaaacggccaatactcatggattatcaa

SEQ ID NO: 710 - DNA, 39 bp, Artificial Sequence
  Primer
catgagtattggccgtttccgtctgctgcaagaacttta

SEQ ID NO: 711 - DNA, 40 bp, Artificial Sequence
  Primer
ttcttgcagcagacgaatcaggccaatactcatggattat

SEQ ID NO: 712 - DNA, 40 bp, Artificial Sequence
  Primer
tgagtattggcctgattcgtctgctgcaagaactttaacg

SEQ ID NO: 713 - DNA, 38 bp, Artificial Sequence
  Primer
atcgaatgggccgtagcgaataacatggatgtaatcaa

SEQ ID NO: 714 - DNA, 40 bp, Artificial Sequence; identical to SEQ ID NO: 73
  Primer

SEQ ID NO: 715 - DNA, 38 bp, Artificial Sequence
  Primer
gttgataaagctgttaaatctggtgtcgtcgtagtagc

SEQ ID NO: 716 - DNA, 38 bp, Artificial Sequence
  Primer
gacgacaccagatttaacagctttatcaactgctgctt

SEQ ID NO: 717 - DNA, 39 bp, Artificial Sequence
  Primer
gataaagctgttgcagatggtgtcgtcgtagtagcggca

SEQ ID NO: 718 - DNA, 40 bp, Artificial Sequence
  Primer
tactacgacgacaccatctgcaacagctttatcaactgct

SEQ ID NO: 719 - DNA, 38 bp, Artificial Sequence
  Primer
aatgagggaacaaaaggatcatcgagtaccgtcggtta

SEQ ID NO: 720 - DNA, 40 bp, Artificial Sequence
  Primer
acggtactcgatgatccttttgttccctcattcccagctg

SEQ ID NO: 721 - DNA, 39 bp, Artificial Sequence
  Primer
aacatccggatcaaaaagtaccgtcggttatccaggcaa

SEQ ID NO: 722 - DNA, 39 bp, Artificial Sequence
  Primer
ataaccgacggtactttttgatccggatgttccctcatt

SEQ ID NO: 723 - DNA, 40 bp, Artificial Sequence
  Primer
tgttgcatctggtccagtcgtagtagcggcagctgggaat

SEQ ID NO: 724 - DNA, 40 bp, Artificial Sequence
  Primer
tgccgctactacgactggaccagatgcaacagctttatca

SEQ ID NO: 725 - DNA, 38 bp, Artificial Sequence
  Primer
agggaacatccggaccatcgagtaccgtcggttatcca

SEQ ID NO: 726 - DNA, 40 bp, Artificial Sequence; identical to SEQ ID NO: 113
  Primer

SEQ ID NO: 727 - DNA, 40 bp, Artificial Sequence
  Primer
cttcaaatcaacgtgactctttttcctccgtgggaccgga

SEQ ID NO: 728 - DNA, 40 bp, Artificial Sequence
  Primer
acggaggaaaaagagtcacgttgatttgaagagtctacag

SEQ ID NO: 729 - DNA, 40 bp, Artificial Sequence
  Primer
tcaacgtgcctctgattcctccgtgggaccggagctggat

SEQ ID NO: 730 - DNA, 37 bp, Artificial Sequence
  Primer
tcccacggaggaatcagaggcacgttgatttgaagag

SEQ ID NO: 731 - DNA, 38 bp, Artificial Sequence
  Primer
tactatggaaaaggggtaatcaacgtacaggcggcagc

SEQ ID NO: 732 - DNA, 38 bp, Artificial Sequence
  Primer
ctgtacgttgattaccccttttccatagtagaaagaat

SEQ ID NO: 733 - DNA, 36 bp, Artificial Sequence
  Primer
tggcgtttctattgaatcgacgcttccagggaacaa

SEQ ID NO: 734 - DNA, 37 bp, Artificial Sequence
  Primer
ctggaagcgtcgattcaatagaaacgccaggggccat

SEQ ID NO: 735 - DNA, 36 bp, Artificial Sequence
  Primer
cttccagggaacacatatggtgcgcaaaacgggact

SEQ ID NO: 736 - DNA, 38 bp, Artificial Sequence
  Primer
gttttgcgcaccatatgtgttccctggaagcgtcgatt

SEQ ID NO: 737 - DNA, 36 bp, Artificial Sequence
  Primer
cttccagggaacctttatggtgcgcaaaacgggact

SEQ ID NO: 738 - DNA, 38 bp, Artificial Sequence
  Primer
gttttgcgcaccataaaggttccctggaagcgtcgatt

SEQ ID NO: 739 - DNA, 40 bp, Artificial Sequence
  Primer
tttctactatggaaacgggctgatcaacgtacaggcggca

SEQ ID NO: 740 - DNA, 40 bp, Artificial Sequence
  Primer
acgttgatcagcccgtttccatagtagaaagaatcaccaa

SEQ ID NO: 741 - DNA, 39 bp, Artificial Sequence
  Primer
tttctaagcacccgaaatggacaaacactcaagtccgca

SEQ ID NO: 742 - DNA, 38 bp, Artificial Sequence
  Primer
gagtgtttgtccatttcgggtgcttagaaagaatcaat

SEQ ID NO: 743 - DNA, 39 bp, Artificial Sequence
  Primer
ttctttctaagcaccgtaactggacaaacactcaagtcc

SEQ ID NO: 744 - DNA, 38 bp, Artificial Sequence
  Primer
tgtttgtccagttacggtgcttagaaagaatcaatgcg

SEQ ID NO: 745 - DNA, 36 bp, Artificial Sequence
  Primer
cacccgaactggcgtaacactcaagtccgcagcagt

SEQ ID NO: 746 - DNA, 40 bp, Artificial Sequence
  Primer
tgcggacttgagtgttacgccagttcgggtgcttagaaag

SEQ ID NO: 747 - DNA, 33 bp, Artificial Sequence
  Primer
cgtctgcttacctctacgccgttaaagttcttg

SEQ ID NO: 748 - DNA, 40 bp, Artificial Sequence
  Primer
actttaacggcgtagaggtaagcagacggggctacaccaa

SEQ ID NO: 749 - DNA, 36 bp, Artificial Sequence
  Primer
agcctgggagcacaaagcggcagtgcggcacttaaa

SEQ ID NO: 750 - DNA, 34 bp, Artificial Sequence
  Primer
cactgccgctttgtgctcccaggctcatgttgat

SEQ ID NO: 751 - DNA, 41 bp, Artificial Sequence
  Primer
ttcaatcgacgcttccaacgaacaagtatggtgcgcaaaac

SEQ ID NO: 752 - DNA, 39 bp, Artificial Sequence
  Primer
caccatacttgttcgttggaagcgtcgattgaatagaaa

SEQ ID NO: 753 - DNA, 39 bp, Artificial Sequence
  Primer
tggattatcaacggcgtagaatgggccatcgcgaataac

SEQ ID NO: 754 - DNA, 39 bp, Artificial Sequence
  Primer
cgatggcccattctacgccgttgataatccatgagtatt

SEQ ID NO: 755 - protein, 269 aa, Bacillus lentus
AQSVPWGISRVQAPAAHNRGLTGSGVKVAVLDTGISTHPDLNIRGGASFVPGEPSTQDGNGHGTHVAGTIAALNNSIGVLGVAPSAELYAVKVLGASGSGSVSSIAQGLEWAGNNGMHVANLSLGSPSPSATLEQAVNSATSRGVLVVAASGNSGAGSISYPARYANAMAVGATDQNNNRASFSQYGAGLDIVAPGVNVQSTYPGSTYASLNGTSMATPHVAGAAALVKQKNPSWSNVQIRNHLKNTATSLGSTNLYGSGLVNAEAATR

SEQ ID NO: 756 - DNA, 1143 bp, Bacillus lentus
gtgagaagcaaaaaattgtggatcgtcgcgtcgaccgcactactcatttctgttgctttcagttcatcgatcgcatcggctgctgaagaagcaaaagaaaaatatttaattggctttaatgagcaggaagctgtcagtgagtttgtagaacaagtagaggcaaatgacgaggtcgccattctctctgaggaagaggaagtcgaaattgaattgcttcatgaatttgaaacgattcctgttttatccgttgagttaagcccagaagatgtggacgcgcttgagctcgatccagcgatttcttatattgaagaggatgcagaagtaacgacaatggcgcaatcagtgccatggggaattagccgtgtgcaagccccagctgcccataaccgtggattgacaggttctggtgtaaaagttgctgtcctcgatacaggtatttccactcatccagacttaaatattcgtggtggcgctagctttgtaccaggggaaccatccactcaagatgggaatgggcatggcacgcatgtggccgggacgattgctgctttaaacaattcgattggcgttcttggcgtagcgccgagcgcggaactatacgctgttaaagtattaggggcgagcggttcaggttcggtcagctcgattgcccaaggattggaatgggcagggaacaatggcatgcacgttgctaatttgagtttaggaagcccttcgccaagtgccacacttgagcaagctgttaatagcgcgacttctagaggcgttcttgttgtagcggcatctggaaattcaggtgcaggctcaatcagctatccggcccgttatgcgaacgcaatggcagtcggagctactgaccaaaacaacaaccgcgccagcttttcacagtatggcgcagggcttgacattgtcgcaccaggtgtaaacgtgcagagcacatacccaggttcaacgtatgccagcttaaacggtacatcgatggctactcctcatgttgcaggtgcagcagcccttgttaaacaaaagaacccatcttggtccaatgtacaaatccgcaatcatctaaagaatacggcaacgagcttaggaagcacgaacttgtatggaagcggacttgtcaatgcagaagctgcaactcgttaa

SEQ ID NO: 757 - protein, 380 aa, Artificial Sequence
  Mutant of Bacillus lentus subtilisin
VRSKKLWIVASTALLISVAFSSSIASAAEEAKEKYLIGFNEQEAVSEFVEQVEANDEVAILSEEEEVEIELLHEFETIPVLSVELSPEDVDALELDPAISYIEEDAEVTTMAQSVPWGISRVQAPAAHNRGLTGSGVKVAVLDTGISTHPDLNIRGGASFVPGEPSTQDGNGHGTHVAGTIAALNNSIGVLGVAPSAELYAVKVLGASGSGSVSSIAQGLEWAGNNGMHVANLSLGSPSPSATLEQAVNSATSRGVLVVAASGNSGAGSISYPARYANAMAVGATDQNNNRASFSQYGAGLDIVAPGVNVQSTYPGSTYASLNGTSMATPHVAGAAALVKQKNPSWSNVQIRNHLKNTATSLGSTNLYGSGLVNAEAATR

SEQ ID NO: 758 - DNA, 27 bp, Artificial Sequence
  Primer
cgcgcttgagctcgatccagcgatttc

SEQ ID NO: 759 - DNA, 25 bp, Artificial Sequence
  Primer
gtctccaagctttaacgagttgcag

SEQ ID NO: 760 - DNA, 30 bp, Artificial Sequence
  Primer
gcaattcagatcttccttcaggttatgacc

SEQ ID NO: 761 - DNA, 30 bp, Artificial Sequence
  Primer
gcatcgaagatctgattgcttaactgcttc

SEQ ID NO: 762 - DNA, 1143 bp, Artificial Sequence
  Mutant of Bacillus lentus subtilisin
gtgagaagcaaaaaattgtggatcgtcgcgtcgaccgcactactcatttctgttgcttttagttcatcgatcgcatcggctgctgaagaagcaaaagaaaaatatttaattggctttaatgagcaggaagctgtcagtgagtttgtagaacaagtagaggcaaatgacgaggtcgccattctctctgaggaagaggaagtcgaaattgaattgcttcatgaatttgaaacgattcctgttttatccgttgagttaagcccagaagatgtggacgcgcttgaactcgatccagcgatttcttatattgaagaggatgcagaagtaacgacaatggcgcaatcagtgccatggggaattagccgtgtgcaagccccggctgcccataaccgtggattgacaggttctggtgtaaaagttgctgtcctcgatacaggtatttccactcatccagacttaaatattcgtggtggcgctagctttgtaccaggggaaccatccactcaagatgggaatgggcatggcacgcatgtggccgggacgattgctgctctaaacaattcgattggcgtacttggcgtagcgccgagcgcggaactatacgctgttaaagtattaggggcgagcggtgggggcgccatcagctcgattgcccaaggattggaatgggcagggaacaatggcatgcacgttgctaatttgagtttaggaagcccttcgccaagtgccacacttgagcaagctgttaatagcgcgacttctaggggcgttcttgttgtagcggcatctggaaattcgggtgcagactcaatcagctatccggcccgttatgcgaacgcaatggcagtcggagctactgaccaaaacaacaaccgcgccagcttttcacagtatggcgcagggcttgacatcgtcgcaccaggtgtaaacgtgcagagcacatacccaggttcaacgtatgccagcttaaacggtacatcgatggctactcctcatgttgcaggtgcagcagtccttgttaaacataagaacccatcttggtccaatgtacgaatccgcgatcatctaaagaaaacggcaacgagcttaggaagcacgaacttgtatggaagcggacttgtcaatgccgaagctgcaactcgttaa

SEQ ID NO: 763 - protein, 380 aa, Artificial Sequence
  Mutant of Bacillus Lentus subtilisin
VRSKKLWIVASTALLISVAFSSSIASAAEEAKEKYLIGFNEQEAVSEFVEQVEANDEVAILSEEEEVEIELLHEFETIPVLSVELSPEDVDALELDPAISYIEEDAEVTTMAQSVPWGISRVQAPAAHNRGLTGSGVKVAVLDTGISTHPDLNIRGGASFVPGEPSTQDGNGHGTHVAGTIAALNNSIGVLGVAPSAELYAVKVLGASGGGAISSIAQGLEWAGNNGMHVANLSLGSPSPSATLEQAVNSATSRGVLVVAASGNSGADSISYPARYANAMAVGATDQNNNRASFSQYGAGLDIVAPGVNVQSTYPGSTYASLNGTSMATPHVAGAAVLVKHKNPSWSNVRIRDHLKKTATSLGSTNLYGSGLVNAEAATR

SEQ ID NO: 764 - DNA, 1140 bp, Artificial Sequence
  Mutant of Bacillus Lentus subtilisisn
gtgagaagcaaaaaattgtggatcgtcgcgtcgaccgcactactcatttctgttgcttttagttcatcgatcgcatcggctgctgaagaagcaaaagaaaaatatttaattggctttaatgagcaggaagctgtcagtgagtttgtagaacaagtagaggcaaatgacgaggtcgccattctctctgaggaagaggaagtcgaaattgaattgcttcatgaatttgaaacgattcctgttttatccgttgagttaagcccagaagatgtggacgcgcttgaactcgatccagcgatttcttatattgaagaggatgcagaagtaacgacaatggcgcaatcagtgccatggggaattagccgtgtgcaagccccggctgcccataaccgtggattgacaggttctggtgtaaaagttgctgtcctcgatacaggtatttccactcatccagacttaaatattcgtggtggcgctagctttgtaccaggggaaccatccactcaagatgggaatgggcatggcacgcatgtggccgggacgattgctgctctaaacaattcgattggcgtacttggcgtagcgccgagcgcggaactatacgctgttaaagtattaggggcgagcggtgggggcgccatcagctcgattgcccaaggattggaatgggcagggaacaatggcatgcacgttgctaatttgagtttaggaagcccttcgccaagtgccacacttgagcaagctgttaatagcgcgacttctaggggcgttcttgttgtagcggcatctggaaattcgggtgcagactcaatcagctatccggcccgttatgcgaacgcaatggcagtcggagctactgaccaaaacaacaaccgcgccagcttttcacagtatggcgcagggcttgacatcgtcgcaccaggtgtaaacgtgcagagcacatacccaggttcaacgtatgccagcttaaacggtacatcgatggctactcctcatgttgcaggtgcagcagtccttgttaaacaaaagaacccatcttggtccaatgtacgaatccgcgatcatctaaagaatacggcaacgagcttaggaagcacgaacttgtatggaagcggacttgtcaatgccgaagctgcaactcgt

SEQ ID NO: 765 - protein, 380 aa, Artificial Sequence
  Mutant of Bacillus lentus subtilisin
VRSKKLWIVASTALLISVAFSSSIASAAEEAKEKYLIGFNEQEAVSEFVEQVEANDEVAILSEEEEVEIELLHEFETIPVLSVELSPEDVDALELDPAISYIEEDAEVTTMAQSVPWGISRVQAPAAHNRGLTGSGVKVAVLDTGISTHPDLNIRGGASFVPGEPSTQDGNGHGTHVAGTIAALNNSIGVLGVAPSAELYAVKVLGASGGGAISSIAQGLEWAGNNGMHVANLSLGSPSPSATLEQAVNSATSRGVLVVAASGNSGADSISYPARYANAMAVGATDQNNNRASFSQYGAGLDIVAPGVNVQSTYPGSTYASLNGTSMATPHVAGAAVLVKQKNPSWSNVRIRDHLKNTATSLGSTNLYGSGLVNAEAATR